European Patent Application EP 4 644 557 A1, published November 5, 2025. Title: RNA-GUIDED ENDONUCLEASE SYSTEM AND USE THEREOF IN GENE EDITING. Applicant: HARBIN INSTITUTE OF TECHNOLOGY. Application EP. The sequence listing filed with the application follows.

SEQUENCE LISTING (233 sequences)

SEQ ID NO: 1 - protein, 387 aa, Catenibacterium sp.
MRKLLKSFKTEINPTEEQKVRIRKTIGTCRFIYNFYLAHNKELHESGKKFMSSSQFRVWLNNEYLPSHPEYSWIKEAYSKSVTQAVNDGQTAFTRFFNHKSAFPKFKKKGKSDVKMYFVRNNPKDCSCERHRIKIPSLGWVRIKEKGYIPTTKDGYVIKSGHVSIKADRYYVSVLIEIPDKTSASNSSEGIGIDLGLKDFAIASNGKTYKNINKSAKLKKLEKKLIREQRSLSRKYENIKKGGSTQKRNIQKQRLKIQKLHHRIDNIRTDYINKIIAEIVKTKPSYITIEDLNISGMMKNRHLSKAVASQKFYEFKTKLQAKCRENGIELRVVDRWFPSSKTCHCCKSIKKDLKLSDRLFRCDCGYIEDRDFNAALNLRDATTYEVA

SEQ ID NO: 2 - protein, 402 aa, Mitsuokella sp.
MKRLLKSFKTELRLTESQTDKVRRSLGICRFLANQYIARNIWLCRLYQRGVLDEKQPHFITANDFDKYVNHVLKKKFPWIDQCGSKARKKVLVNAEQAFRRFFKGPARFPRFKRKNQQNVKLYFPKNNKGDWTIWRHKIQIPTIGRVRLKEFGYLPQGVTIKNGHVSCEAGRYYVSVTAEIEETSRYNNDLEASYHPQSDGIGVDLGVKSLAIVSDGRIFENINTSSRARRLEKRLRREQRRLSRKYEIRKKKGGSTATASANIEKKRLSVQKLHQRLTNLRRNYENQVIHALVEQKPRFITMEDLNVTGMMKNRHLSKSVAQQRFYSLREKLRRKAEIIGIEFRIADRFYPSSKTCHACGHVHGGLKLKDRIYVCPVCGYTEDRDLNAALNLRDTKNYRIA

SEQ ID NO: 3 - protein, 387 aa, Blautia sp.
MRKLQKSFKTEINPTDEQKLKIRRTIGTCRYVYNFYLDQNRKRYEKGEKFMSGKSFSVWLNNEYLPQNPEYAWIKEVSSKSVKRSLENACTAFSRFFKGQSHFPRYKKKNKSNVKMYFVKNNRTDCFCERHRVNIPTLGWVRIKEKGYLPTTKDGYVIKSGTVSMRAGRYYVSVLVEVPDPPKEENRNEGIGIDLGIKSFAVLSDGTVYQNINKSAKIKKLEKQLRREQRSLSRKYENLKKGVSTQRANIQKQKLKVQRLYQRIDNIRTDYIKKTIAGIVKTKPSFVTIEDLNVKGMMKNRHLSKATASQKFYEFRTRLQGKCAEKGIELRIADRWYPSSRRCHNCGQIRKDLKLSNRVYQCSCGYCEDRDLNAALNLRDVKTYQSA

SEQ ID NO: 4 - protein, 387 aa, Ruminococcus sp.
MRRLLKSFKTEIDPTEEQKIKIHKTIGTCRYIYNFYLFHNKERYDAGERFMSGKSFSVWLNNEYLPGHPEYFWIREVSSKSVKNTIENACTAFSRFFHHQSSFPRYKKKGRSDVKMYFVKNNPKDCLCERHRIKIPTLGWVRLKEKGYIPASKDGFVIRSGAVSMKAGRYYVSALVDIPAPEADGNFTDGIGIDLGLKDFAVVSNGTVYRNINKTARIRKLEKQLRRAQRKLSRKYENLKKGESTQRANICKQKLKVQKLHHRIENIRTDHINKVISEIVKTKPSHITIEDLNISGMMKNRHLSKAVASQKFYEFRTKLKIKCAEYGIELRVVDRWYPSSRICHCCSCIKKDLKLSDRIYRCTCGYIEDRDLNAARNLRDAETYEVA

SEQ ID NO: 5 - protein, 387 aa, Clostridium sp.
MWKLLKSFKTEINPTEEQKVKIRKTIGTCRYIYNFYLAHNKELHDNGKKFMSGKSFSVWLNNEYLPQNPDKLWIKEVSSKSVKRSIENGCVAFTRFFKHQSAFPNFKKKGKSDVKMYFVKNNPKDCRCERHRINIPSLGWVRIKEKGYIPTTKDGYVIKSGTVSIKAGRYYVSVLVEIPDMLIDSSNNDGIGIDLGLKNFAIVSNGKTYKNINKSARLKKLEKQLRREQKCLSRKYEYLKKGESTQRANIQKQKLKVQKLYHRLDNIHTDYINKIIAEIVKTKPSYITIEDLNVSGMMKNRHLSKAVASQKFYEFRTTLKSKCDDNNIELRVVDRFYPSSKLCHCCGSIKKDLKLSDRIYRCDCSYVADRDLNAALNLKDAKTYKIA

SEQ ID NO: 6 - protein, 387 aa, Firmicutes bacterium
MWKLLKSFKTEINPSEEQKVKIHKTIGTCRFIYNFYLAHNKELYDKGEKFMSGKSFSVWLNNEYLPQNPDKLWIKEVSSKSVKHSIENGCIAFTRFFKHQSAFPNLKKKGKSDVKMYFVKNNPKDCRCERHRINIPSLGWVRIKEKGYIPTTKDGYVIKSGTVSMKADRYYVSVLVEISNNKIANNSNAGIGIDLGLKDFAIVSNGKTYKNINKSARLKKHEKQLIREQRSLSRKYENLKKGESTQKANIQKQRLKVQKLHHRMDNIRTDYINKTIAEIVKTKPSYITIEDLNVKGMMKNRHLSKAVASQKFYEFRTKLQAKCNENGIELRVVDRWYPSSKTCHCCGAVKKDLKLSDRIFKCSCGYVEDRDFNAALNLRDAITYEVA

SEQ ID NO: 7 - protein, 387 aa, Lachnospira sp.
MRKLLKSFKTEINPTEEQKAKIRKTIGTCRYIYNFYLAHNKELYNKGEKFMSSNQFRVWLNNEYLPKHPECFWIKEAYSKAVTQAVNNGQAAFIRFFKHQSSFPRFKKKNRSDVKMYFVKNNPKDCRCQRHRINIPSLGWVRIKEKGYIPTTKDGYVIKSGHVSIKAGRYYVSALVEIPNNKIANSFNEGIGIDLGIKDFAIVSNGKIYKNINRSVRLKKLGKQLIREQKNPSRKYENLKKGESTQKANIQKQRLKVQKLHHKIDNIRTDHINKTIAEIVKTKPSYITIEDLNISGMMKNKHLSKAVASQKFYEFRIKLQAKCNENGIELRVVDRWYPSSKTCHCCGAIKKDLKLSDRIFKCDCGYSEDRDFNAALNLRDATTYEIA

SEQ ID NO: 8 - protein, 387 aa, Dorea formicigenerans
MWKLLKSFKTEINPSEEQKVKIHKTIGTCRFIYNFYLAHNKELYDNGEKFMSSNKFRVWLNHEYLSEHPEYSWIKEVYSKAVTQAVNNGQTAFARFFNHESAFPNFKKKGKSDVKMYFVKNNPKDCRCERHRINIPSLGWVRIKEKGYIPTTKDGYVIKSGTVSMKADRYYVSVLVEILNNKIANNSNAGIGIDLGLKEFAIVSNGKTYKNINKSARLKKLEKQLIREQRSLSRKYENLKKGESTQKTNIQKQRLKVQKLHHRIDNIRTDYINKTIVEIVKTKPSYITIEDLNVKGMMKNRHLSKAVASQKFYEFRTKLQAKCNENGIELRVVDRWYPSSKTCHCCGAVKKDLKLSDRIFKCSCGYVEDRDFNAALNLRDAITYEVA

SEQ ID NO: 9 - protein, 387 aa, Eubacterium hallii
MARLLKSFKTEINPSEEQKVRIYKTIGTCRFIYNFYLSHNKELYDKGEKFMSSNKFRLWLNNEFLPDNPDKMWIKEAYSKAVTQAVNHAQTAFKKFFDHKTAFPRFKKKGKSDVKMYFVRNNPKDCRCERHRIHIPSLGWIRIKEKGYIPTTKDGYIIKSGTVSIKAGRFYVSALVEVPDRKITEPFNEGIGIDLGLKEFAVVSNGRIYKNINRSARIRKLEKQLIREQRRLSRKYEDLKKGETTQKANIQKQKRKVQKLHQRIQNIRTDYMNKIIAEIVKTKPSYITIEDLNVKGMMKNRHLSKAVASQKFYEFRRKLQAKCTEKGMELRIADRWYPSSKKCHCCGCINKELKLSDRIYRCGCGYVEDRDFNAALNLRDARTYKTA

SEQ ID NO: 10 - protein, 387 aa, Clostridiaceae bacterium AF18-31LB
MRKLLKSFKTEINPTEEQKTKIRKTIGTCRFIYNFYLAHNKKLHEDGKKFMSSNKFRIWLNNEYLPQHPEYLWIKEAYSKAVTQSVNNGQTAFTRFFNHESAFPNFKKKGKSDVKMYFVKNNPKDCHCERHRIKIPSLGWVRIKEKGYIPTTKDGYVIKSGSVSIKADRYYVSVLVEVSDNKTINHFDEGIGIDLGLKDFAIVSNGRTYQNINKSAKLKKLERQLIREQRCLSRKYENLKKGDATQRANIQKQKLKVQKLHHRIDNIRTDYINKTIAEMVKIKPSYITIEDLNVKGMMKNRHLSKAVASQKFYEFRAKLLTKCNKSGIELRVVDRWYPSSKICHCCGSIKKDLKLSDRIFKCRCGYIEDRDFNASLNLRDAETYSIA

SEQ ID NO: 11 - protein, 386 aa, Roseburia inulinivorans
MRKLLKSFKTEINPTVEQKIKINKTIGTCRYVYNFYLGHNKALYDKGEKFMTGKSFSVWLNNEYIPNNPDKIWIKEAYSKAVKKSIEDGCTAFTRYFKHQSAFPNFKKKGKSDVKMYFVKNNPKDCRCERHKLNIPTLGWVRMKEKGYIPTTKDGWKIKSGTVSIKADRYYVSVLVEIPDAKITDNSNDGMGIDLGLKDLAIVSNGKTYKNINKSARVKKLEKKLRREQRCLSRKYENLKKGESTQKNIQKQKLKVQRLHHKIDNIRTDYINKSIAEIVKAKPSYITIEDLNVSGMMKNRHLSKAVASQKFYEFRTKLKAKCDENGIELRVVDRWYPSSKICHCCGAVKKDLKLSDRIYRCDCGYIEDRDFNAALNLRDALTYEVA

SEQ ID NO: 12 - protein, 387 aa, Anaerobutyricum hallii
MRKLLKSFKTEIDPTEEQKVRIHKTIGTCRFIYNFYLAHNKELHKNGERFMSSSKFRVWLNNEYLPNHPEYSWIKEAYSKAVTQAVNNGQTAFTRFFNHESNFPNFKKKGRSDVKMYFVKNNPKDCCCERHRIKIPSLGWVRIKEKGYIPTTKDEYVIKSGHVSIKADRYYVSVLVEIPDDKMVNNSNEGIGIDLGLKDLAIISNGKTYKNINKSAKLKKLEKQLIRGQRSLSRKYENSKKGESTQRANIQKQKIKVQKLYQKIDNIRTDYINKTIAEIVKTKPSFITIEDLNVKGMMKNRHLSKAVASQKFYEFRIKLQAKCNENGIELRVVDRWYPSSKTCHCCKNIKKDLRLSDRIFKCDCGYIEDRDLNAALNLRDAMTYEVA

SEQ ID NO: 13 - protein, 386 aa, Eubacterium rectale
MRKLLKSFKTEINPTIEQKIKINKTIGTCRYVYNFYLGHNKTLYDNGEKFMTGKSFSVWLNNEYIPNNPDKIWIKEAYSKAVKKSIEDGCTAFTRFFKHQSAFPNFKKKGKSDVKMYFVKNNTKDCRCERHRLNIPTLGWVRIKEKGYIPTTKDGWKIKSGTVSVKADRYYVSVLVEIPNVKIANNSNGGIGIDLGLKDLAIVSNGKTYKNINKSTRIKKLEKKLRREQRCLSRKYENLKKGESTQKNIQKQKLKVQRLHHKIDNIRTDYINKSIAEIVKTKPSYITIENLNVSGMMKNRHLSKAVASQKFYEFRTKLKAKCDENGIELRVVDRWYPSSKICHCCGAIKKDLKLSDRIYRCDCGYVEDRDFNAALNLRDALTYEVA

SEQ ID NO: 14 - protein, 385 aa, Bacillus cereus
MKRAYLIEIKPTTEQVSKIHQTIGVCRYVYNLYISKNKEAYESEGKFLSGYDFSKWLNNIHTKECDQWIKEVSSKAVKQAIMNGDKAFKRFFKGLSKFPRYKKKRKQDVKCYFPKNNKTDWTVERHRVKVPTIGWVRLKEYGYIPKNATVKSGTVYQRAGRYFVSVLCERAEIRVKPMLNKVGLGIDLGLKDFAVRSDGKTHKNINKTVQVKKIEKRLKREQRSLSRKFENRKKRGEQSVTNKRANIDKNILRVQKLHARLANIRLAYVKSIVNDVVKTKPTFITVEDLNVKGMMKSKHLSKTIAKQSFFAFKTWLLTKCEEYGIELRQVDRFYPSSKLCSCCSQKKVDLKLSDRVYTCECGNVMDRDLNAAINLLQAKEYTILT

SEQ ID NO: 15 - protein, 370 aa, Weizmannia coagulans
MILAKKVRLNPTEEQERQLWKSVGTARWVYNWTLSKQEESYKNDGKFISDGELRKELTQLKKTEEYSWLLDVSNNVAKQAVKDACDAYKKFFKKLANKPRFKSRKRSKPSFYNDNVKLKVKEMLVLIEKVGWVKTSEQLPINTKYVNPRVSFDGKYWYLSVGIQQKHVHNDLTDNIIGIDVGVKELAVCSNGMVFKNINKTKTVKKIEKRLRRLQRKVSRKYEMNKEGNRFVKTCNIIKTEKKIRLLHRRLMNIRTNHIHQTTNAIVKTKPSTVVMEKLNIKGMMKNKYLSKAVQNQKLYEFKRQMKYKCEFNGIKFIEADKWYPSSKTCSNCGQIKKDLKLSERIFRCDCGLEIDRDLNASINLAKLAN

SEQ ID NO: 16 - protein, 387 aa, Blautia sp.
MVKAIKVMLIPNNVQKTKMFQYAGASRFAYNWALAREKENYEKGGRFIPDAELRKEFTKLRHSDEYAWLLSISNNVTKQAIKDACTAYKNFFKGLQKFPRFKYRKRSMPKFYQDNVKIRFSNTHVKFEGFSSGRKANKQKMNWVRLAEHGRIPTDAKYMNPRISFDGLNWWISVCVELPDCRETPNDDGVGIDLGIKNLAVCSDAVKYKNINKSQKVKKLEKQKRGLQRSISRSYEKNKRGESYCKTNNVIKKKKLLLKRNHRLTNIRKNYLNQTISEIVNRKPRFICIEDLNVSGMMKNRHLSKAVQEQGFFRFRKQLEYKCSDKGIQLIVADRFYPSSKLCSCCGNIKKDLKLSDRIYRCECGNRIDRDFQASINLKIYGERFAS

SEQ ID NO: 17 - protein, 384 aa, Blautia sp.
MLKSFKTEIHPTEEQKVRIHKTIGTCRFIYNFYLAHNKELYQNGEKFMSSSKFRVWLNHEYLPQHPEYLWIKEAYSKAVTQAVNHGQTAFKKFFNHESAFPKFKKKGRSDVKMYFVKNNPKDCRCERHRVNIPSLGWVRIKEKGYIPTTKEGYIIKSGHVSMKAGRYYVSALIEIPDNKTADLSNEGIGIDLGLKDFAIVSNGKTYKNINKSARLKKLEKRLVREQRCLSRKYENLKKGESTQRANIQKQKLKVQKLHHKIDNIRTDYINKTIAEIVKTKPSYITIEDLNVSGMMKNKHLSRAVASQKFYEFRIKLKAKSRENGIELRVADRWYPSSKICHCCGTIKKDLKLSDRTFRCHCGYVEDRDFNAALNLRDVKTYKIA

SEQ ID NO: 18 - protein, 387 aa, Blautia sp.
MRRLLKSFKTEINPTEEQKIKIHKTIGTCRYIYNFYLFHNKERYDIGEKFMSGRAFSVWLNNEYLPKHPEYSWIREVSSKSVKNAIENACTAFSRFFHHQSGFPRYKKKGRSDVKMYFVRNNPKDCFCERHRIKIPTLGWVRLKEKGYIPTSRDGYVVRSGAVSMKAGRYYVSALIEVPTPKVDGNFSDGIGIDLGLKNFAVVSNGTVYRNINKTVQIRKLEKQLTRAQRKLSRKYENLRKGEFTQKANIQKQKLKVQKLYDRIENIRTDHINKTISEIVKTKPSHITIEDLNVSGMMKNRHLSKAVSSQKFYEFRTKLKAKCAEYGIELRVVDRWYPSSKTCHCCGCIKKDLKLSDRIYKCTCGYVEDRDFNAALNLRDARTYKVA

SEQ ID NO: 19 - protein, 386 aa, Butyricicoccus sp.
MRELLKSFKTEINPTAEQKVKINKTIGTCRFVYNFYLDHNKALHNKGEKFMTGKSFSVWLNNEYIPNNPDKAWIKEAYSKAVKKSIENGCIAFTRFFKHQSAFPNFKKKGKSDVKMYFVKNNPKDCRCERHRLNIPTLGWVRIKEKGYIPTTKDGWRIRSGTISIKAGRYYVSVLIEVPDVKNTNNNSKGIGIDLGLKDFAIISNGKIYKNINKSARVKKLENKLRREQRCFSRKYENLKKGESTQKNIQKQELKVQRLHHKIVNIRTDYINKTIAEIVKTKPSYITIEDLNVSGMMKNKHLSKAVASQKFYEFRTKLKAKCDENGIELRIVNRWYPSSKICHCCGAIKKDLKLSDRIYRCGCGYVEDRDFNAALNLRDALTYEIA

SEQ ID NO: 20 - protein, 386 aa, Clostridiaceae bacterium AF18-31LB
MKKLLKSFKTEINPTVEQKIKINKTIGTCRYVYNFYLVHNRNLHDQCEKFMTGKSFSVWLNNEYIPNHPDKAWIKEAYSKAVKKSIEDGCTAFTRFFKHQSDFPNFKKKGKSDVKMYFVKNNPKDCRCERHRLNIPTLGWVRIKEKGYIPTTKDGWKIKSGTVSIRAGRYYVSALVEVPDATIYNNNNDGVGIDLGLKDLAIVSNGKTYKNINKSARVKKLEKQLRREQRCLSRKYESLKKGESTQKNIQKQKRKVQKLHHKIDNIRTDYINKTVAEIVKTKPSYITIEDLNISGMMKNRHLSKAIASQKFYEFRIKLKAKCDENGVELRVADRWYPSSKICHCCGTIKRDLKLSDRIYRCSCGYIEDRDFNASLNLRDAITYKIA

SEQ ID NO: 21 - protein, 387 aa, Clostridiales bacterium AM23-16LB
MRKLLKSFKTEINPTEEQKTKIRKTIGTCRFIYNFYLAHNKKLHEDGKKFMSSNKFRIWLNNEYLPQHPEYSWIKEAYSKAVTQSVNNGQTAFTRFFNHESAFPNFKKKGKSDVKMYFVKNNPKDCHCERHRIKIPSLGWVRIKEKGYIPTTKDGYVIKSGSVSIKADRYYVSVLVEVSDNKTINHFDEGIGIDLGLKDFAIVSNGRTYQNINKSAKLKKLERQLIREQRCLSRKYENLKKGDATQRANIQKQKLKVQKLHHRIDNIRTDYINKTIAEMVKIKPSYITIEDLNVKGMMKNRHLSKAVASQKFYEFRAKLLAKCNESGIELRVVDRWYPSSKTCHCCGSIKKDLKLSDRIFKCRCGYIEDRDFNAALNLRDAETYSIA

SEQ ID NO: 22 - protein, 390 aa, Clostridium perfringens
MKKLKRAYKIEINPTAEQKSKIHQTIGVSRFIYNFYIAHNKEIYAREGKFVSGMDFSKWLNNKYIPNNKDMKWIKEVSSKATKQAIMNGDKAFRDFFKKAKGFPKFKKKKNQDVKAYFPKNNKTDWTLERHKVKIPTLGWVRLKEFGYIPVNSIVKSGTVSQKADKYYVSILVEEDDKKVYKSTNEGLGIDLGVKEFVVCSNGIKFKNINKTSTVKKVEKKLKREQRKLSRKYESLKIRNKNLKEGRATSQNIQKQLVKVQKLHQRLTNIRTDYINKIVSSIIKQKPSYITIEDLAVSNLMKNKHLSKAIASQKFFEFKTKLMFKCKENHIELRIVDRFYPSSKTCSSCGKVKKDLKLSDRVYKCDCGLTIDRDLNASINLKNAKEYKIA

SEQ ID NO: 23 - protein, 387 aa, Coprococcus catus
MVKAIKVMLIPNNVQKTKMFQYAGASRFAYNWALAREKESYEKGGRFISDSELRKEFTKLRHSDEYAWLLNISNNVTKQAIKDACTAYKNFFKGLQKFPRFKSRKRSMPKFYQDNVKIQFSNTHVKLEGFSSSRKANKQKKNWVRLAEHGRIPTDVKYMNPRISFDGLNWWISVCVEFPDCKETLNDDGVGIDLGIKDLAVCSDAVKYKNINKSQKVKKLEKQKRRLQRSISRSYEKNKKGESYCKTNNVIKKEKLLLKRNHRLTNIRKNYLNQTISEIVNRKPRFICIEDLNVSGMMKNRHLSKAVQEQGFFWFRKQLECKCNDKGIQLIVADRFYPSSKLCSCCGNIKEDLKLSDRVYRCECGNMIDRDFQASINLKAYGERFAS

SEQ ID NO: 24 - protein, 387 aa, Coprococcus comes
MVKAIKVMLIPNNVQKTKMFQYAGASRFAYNWALAREKENYEKGGKFISDSELRKEFTKLRHSDEYAWLLNISNNVTKQAIKDACTAYKNFFKGLQKFPRFKSKKRSMPKFYQDNVKIQFSNTHVKFEGFSSSRKANKQKMNWVRLAEHGRIPTDVKYMNPRISFDGLNWWISVCVEFPDCKETLNDDGVGIDLGIKDLAVCSDAVKYKNINKSQKVKKLEKQKRRLQRSISRSYEKNKKGESYCKTNNVIKKEKLLLKRNHRLTNIRKNYLNQTISEIVNRKPRFICIEDLNVSGMMKNRHLSKAVQEQGFFWLRKQLEYKCSDKGIQLIVADRFYPSSKLCSCCGNIKKDLKLSDREYRCECGNIIDRDFQASINLKGYGERFAS

SEQ ID NO: 25 - protein, 392 aa, Coprococcus sp.
MIKSIKVRLCPNNKQLTKLFQYAGCARFAYNWAIAREQENYKQGDKFLSDNELRKEFTQLKKQSEYQWLSEVSNNVTKQAIKDACNTYKKFFKGQCKYPKFKSRKHSSPSFYQDNIKIQFSDTHVKVEGFSMSKKKNKQKLNWIRLCEKGRIPTNCKYMNPRFTYDELHWYISVGIEVEDSTTIPLNNGIGIDLGIKDLAVCSDGNIYKNINKTTTVNKLEKRKRRLQRSISRRYEKNKKGGIYCKTCNIIKKEKELLKVTKRLTNIRQNYLHQTTSEIIKRKPSFICIEDLNVSGMMKNKHLSKAVQQQCFYEFRKQMEYKSAWNNIPVIIADRFFPSSKLCSCCESIKKDLKLSDRIYKCECGNVIDRDYQASLNLKMYGENVLKQQSVA

SEQ ID NO: 26 - protein, 387 aa, Dorea formicigenerans
MVKAIKVMLLPNNVQKTKMFQYAGASRFAYNWALAREKESYEKGGKFISDSELRKEFTKLRHSDEYAWLLNISNNVTKQAIKDACTAYRNFFKGLQKFPRFKSRKRSMPKFYQDNVKIQFSNTHVKLEGFSSSRKANKQKKNWVRLAEHGRIPTDVKYMNPRISFDGLNWWISVCVEFPDCKETLNDDGVGIDLGIKDLAVCSDAVKYKNINKSQKVKKLEKQKRRLQRSISRSYEKNKKGESYCKTNNVIKKEKLLLKRNHRLTNIRKNYLNQTISEIVNRKPRFICIEDLNVSGMMKNRHLSKAVQEQGFFGFRKQLEYKCNDKGIQLIVADRFYPSSKLCSCCGNIKKDLKLSDRVYRCECGNMINRDFQASINLKTYGERFAS

SEQ ID NO: 27 - protein, 311 aa, Dorea formicigenerans
MYSKAVKKSIEDGCAAFTRFFKHQSDFPKFKKKGKSDVKMYFVKNNPKDCQCERHRLKIPTLGWVRIKEKGYIPTTKAGYMIRSGTVSVKAGRFYVSVLVEIPDVNINNNLNEGIGIDLGLKDFAIISNGKTYRNINKSAGLKKLEKQLIREQRSLSRKYENLKKGESTQRANIQKQKLKVQKLHHKMDNIRTDYINKTIAEIVKTKPSYITIEDLNVKGMMKNRCLSKAVASQKFYEFRKRLKAKCDEKGIELRIADRFYPSSKTCHHCGSIRKNLKLSDRIYRCECGYVADRDLNAALNLKDAKTYKIA

SEQ ID NO: 28 - protein, 387 aa, Dorea sp.
MRKLLKSFKTEINPTEEQKVKIRKTIGTCRFIYNFYLAHNKELHKNGEKFMSSNKFRVWLNNEYLPNHPEYSWIKEAYSKAVTQAVNNGQTAFTRFFNHKSSFPNFKKKGKSDVKMYFVKNNPKDCRCERHRINIPSLGWVRIKEKGYIPTTKDGYVIKSGHVSIKADRYYVSVLIEIPNVKIANNSNAGIGIDLGLKDFAIVSNGKTYKNINKSAKLKKLEKQLIREQRSLSRKYENLKKGESAQKPNIQKQRLKVQKLHHRIDNIRTDYINKTIAEIVKTKPSYITIEDLNISGMMKNKHLSKAVASQKFNEFRTKLQAKCNENGIELRVVDRWFPSSKTCHCCKNIKKDLKLSDRIFKCDCGYIEDRDFNAALNLRDATTYEVA

SEQ ID NO: 29 - protein, 402 aa, Firmicutes bacterium
MIKSIKVRLNPNNKQSTKLFQYAGCARFAYNWAISREQDNYKQGNKFLSDSELRKEFTQLKKQSEYQWLNEVSNNVTKQAIKDACNTYKRFFKGQCKYPKFKSKKHSTPSFYQDNIKIQFTDTHVKVESFSMSKKQNKQKLNWIKLCEKGRIPTGCKYMNPRFTYDGLYWYVSIGIEVNDNTTLPSNEGIGIDLGIKHLAICSDGNTYKNINKTQTVKKLEKKKRRLQRSISRKYEKNKKGANYCKTSNIIKREKELLKLNHRLTNVRQNYLHQTTSEIVKREPSFICIEDLNVSGMMKNKHLSKAVQQQGFYEFRRQIEYKAMWNNIPVVIADRFFPSSKLCSCCGSIKKDLKLSDRIYKCECGNVIDRDYQAALNLKQYGENVLKQQSVAYHFQVITDMY

SEQ ID NO: 30 - protein, 387 aa, Firmicutes bacterium
MVKAIKVMLIPNNVQKTKLFQYAGASRFAYNWALAREKENYEKGGKFISDSELRKEFTRLRHSDEYAWLLNISNNVTKQAIKDACTAYQNFFKGLQKFPRFKSRKRSMPKFYQDNVKIQFSNTHVKFEGFSSSRKANKQKRNWVRLAEHGRIPTDAKYRNPRISFDGLNWWISVCVEFPDSKETLNEDGVGIDLGIKDLAVCSDAVKYKNINKSQKVKKLEKQKRRLQRSISRSYEKNKKGESYCKTNNVIKKEKFLLKRNHRLTNIRKNYLNQTISEIVNRKPRFICIEDLNVRGMMKNRHLSKAVQEQGFFGFRKQLEYKCSDKGIQFIVADRFYPSSKLCSCCGNIKKDLKLSDRIYRCECGNRIDRDFQASINLKAYGEQFAS

SEQ ID NO: 31 - protein, 343 aa, Firmicutes bacterium
MVKAIKVMLIPNNVQQTKLFQYAGASRFAYNWALAREKENYEKVGRFIPDTELRKEFTRPRNSDEYAWLLNVSNNVTKQAIKDACSAYKNFFKGLQRYPRFKAKKKSMPKFYQDNIKIQFRDTNVKFEGFSSSRKANKQKLNWVKLAEHGRIPTDAKYRNPRVSFDGLNWWISVCVEFPDCRDRSNHDGIGIDLGIKDLAICSDGNTYKNINKSQTAKKLEKCKRRLQRSVSRKYEHNKKGGSYCKTNNIVKKEKLLLKVNHRLANIRKDYLNQTTSEIANRKPRFICIEDLNVSGMIKNRHLSKAVQNQGFFEFRKQLEYKCNDRDFQASLNLKAYGEQFAS

SEQ ID NO: 32 - protein, 387 aa, Lachnospiraceae bacterium
MVKAIKVMLIPNNVQKTKMFQYAGASRFAYNWALAREKENYEKGGRFISDSELRKEFTKLRHSDEYAWLLSISNNVTKQAIKDACIAYKNFFRGLQKFPRFKSRKRSMPKFYQDNVKIQFSNTHVKFEGFSSSRKANKQKMNWVRLAEHGRIPIDANYMNPRISFDGLNWWISVCVEFPDCRETLNDDGVGIDLGMKDFAVCSDAVKYKNINKSQKVKKLEKQKRRLQRSISRSYEKNKKGESYCKTNHVIKKEKLLLKRNHRLTNIRKNYLNQTVSEIVNRKPRFICIEDLNVSGMMKNRHLSKAVQEQGFFLFRKQLEYKCSDKGIQLIVADRFYPSSKLCSCCGNIKKDLKLSDRVYRCECGNMIDRDFQASINLKAYGERFAS

SEQ ID NO: 33 - protein, 375 aa, Megamonas funiformis
MILAKKVRIYPTKEQEQKLWQSVGTARFIYNYTLAKQEENYKNGGKFISDGIIRKELTQLKKSELIWLNEVSNNVTKQAVKDACNAYKRFFKGLAKKPKFKIRKKSKPSFYNDTSKLKVKEKKVLIEKVGWIKTNEQIPIDVKYNNPRVTYDNKYWYISVGVEVDKKQEELTDISLGIDLGLKDLAVCSDGKVFKNINKTKEVKNLEKRLKQKQRQISRKYEINKIKKGGSCQFIKTKNIEKLENTTKLMHRKLTNIRDNYIHQVTTSIVKTKPYRIVIEDLNVSGMIKNKHLSDSVRKQCFNKFRQYITYKAELYGIGLVIADRFYPSSKTCSECGSIKKDLKLKDRVYRCPHCGVVIDRDYNASLNLSMYKLA

SEQ ID NO: 34 - protein, 377 aa, Megamonas rupellensis
MILAKKVRIYPTKEQEQKLWQSVGTARFIYNYTLAKQEENYKNGGKFINDGVIRKELTQLKKSELTWLNEVSNNITKQSVKDACKAYKRFFKNLANKPKFKSRKKSKPSFYNDPIKLKIKEKKVLIEKVGWIKINEQIPINVKYNNPRITYDNKYWYLSVGIEVDKKQEGLTNISLGIDLGLKELAICSDGKVFKNINKTKKIKKLEKRLKQKQRQISRKYEINKIKKEGGKRYQFIKTKNIKKLENTTKLIYRKLANIRNNYIHQVTTSIVKTKPYRIVIEDLNVSGMMKNKHLSDSVKKQCFHKFRQYITYKSELNGIELVVADRFYPSSKTCSKCGFIKKDLKLKDRVYRCPHCGAVIDRDLNASLNLSMYKLA

SEQ ID NO: 35 - protein, 393 aa, Mitsuokella multacida
MLKAFKTEIAPTKEQRDKIIRSIGVARFLYNQYISYNRRLYKMYRRGMLDERQKYFVTAVDFDKYVNHKLKQELPWIDQCGSKARKKALVNAEQAFRRFFAGISRFPTFKKKTNQDVKLYFPRNNKGDWKIWRHKLMIPTLKQVKLKEYGYLPVGMTATSGTVSYVAGRFYVSVVVDIDAKSKYNKDLDSCYAIQTEGIGIDLGVKDLAVVSDGRVFENINKSSKVKRLEKRLRREQRRLSRKYVGKVDTVSANIEKQKLKVQKLHQRITRIREDYENKTVHEIVKQKPRFITVEDLNVKGMMKNRHLAKAVAAQRFNHLLSKLKRKAKIIGIELREVDRFYPSSKTCHACGHVHRGLKLKDRVYICPECGYRMDRDYNASLNLRDAKEYRVV

SEQ ID NO: 36 - protein, 402 aa, Mitsuokella multacida
MRNLLKSFKTELRLTEGQRDKVRRSLGICRFLANQYIARNIWLYRLYQRGVLDEKQRRFVTANDFDKYVNHVLKKKFPWIDQCGSKARKKILVNAEQAFRRFFRGQAHFPRFKRKNQQNVKLYFPKNNKGDWTIWRHKIQIPTIGKVRLKEFGYLPQGVTIKNGHVSYKAGRYYVSVTAEIEEMSRYNNDLEASYHPRSDGIGVDLGVKSLAIVSDGRIFENINRTSRARRLERRLRREQRRLSRKYEMRKKKGGSTATASANIEKKKLSVQRLHRRLANLRRNHENQVIHALVEQKPRFITVEDLNVTGMMKNRHLSKAVVQQRFYTFREKLRRKAEIIGIEVRIADRFYPSSKTCHACGHVHSGLKLKDRTYVCPACGYKKDRDFNAALNLRDTKNYRIA

SEQ ID NO: 37 - protein, 434 aa, Mitsuokella sp.
MIRSIRVQLLPNNKQKTKLFQFAGAARYAYNWALDKQMDNFREGRKLQTDHELRKAFTLLRHSEENKWLLDISNNVTKQAIKDLCIAYKNFFHKQKQPIYIKYSSKKITHYNRIGKSLTVYDMNGHPKFRSKKNGDFRFYQDNVKIQFTGTHVKLESLAGSRRKNRQRLNWVRLAERNRIPVRAKYTNPRIAFDGERWWLSVGIQTARKLKPLRGLSFVCKKRRYARSEGIGIDLGIKDLAVLSDATKVGNINKTRAIRKLKKKRRRLQRQVSQKYQMNKKGDSYCKTSNLIKSEKRLLRINHRLANIRQNHVHQATTSIIKRKPSFVCLEDLNVRGMMKNRYLSEKIQEQNLYEFRRQIEYKAHWAKIPVVIADRWYPSSKTCVICGHVKKELNLLERTYICPVCGNIIDRDFQAALNLKRYGEAEQVKLANY

SEQ ID NO: 38 - protein, 370 aa, Peptoclostridium sp.
MEKGFKVQIFPNKEQKELMFKSFGCARFAYNWALAKEKENYEKGGKFISDMDLRKEFTQLKKKEEFKWLNEINNNVTKQAIKDLCKAYKNFFKKKAEHPRFKSKKKSKKSFYNDVYKIKFDDYKVRIESIGWMDMAENRIPRNCKYQNPKISFDGVKFWLSITCIVEDEENNLPKTEPIGIDMGIKTLMTCSNGMNFNRVSTKKEKKKLKRLQKKASRHYDKMMKTKSSDKSKNLLKLETLIRKQYQRISNVRLNNIHQATTKLVKLNPKAIVVEDLNVKGMIKNKYLSEKIADCSFYEIYRQLEYKCENKGMEFIVADRFYPSSKICSNCGHKKEKLSLSERTYRCECCGNVIDRDFNASLNLKNLAYN

SEQ ID NO: 39 - protein, 387 aa, Ruminococcus sp.
MVKAIKVMLIPNNIQKTKMFQYAGASRFAYNWALAREIENYEKGGKFISDAELRKEFTKLRHSDEYAWLLSISNNVTKQAIKDACTAYKNFFKGLQKFPRFKPKKRSIPKFYQDNIKIQFSNTHVKFEGFSSSRKRNKQKLNWVRLAEHGRIPTDAKYMNPRISFDGLNWWISVCVEFPDCIEKLNDDGIGIDLGIKDLAICSDGAKYKNINKSQKVKKLEKQKRRLQRSISRSYEKNKKGESYCKTNNVIKKEKLLLKRNHRLTNIRKNYLNQTTSEIVSRKPRFICIEDLNVSGMMKNRHLSKAVQNQGFFEFRKQLEYKCSDKGIQLIVADWFYPSSKLCSCCGNIKKDLKLSDRIYKCDCGNVIDRDFQASINLKAYGERVAS

SEQ ID NO: 40 - protein, 387 aa, Ruminococcus sp.
MWKLLKSFKTEINPSEEQKVKIHKTIGTCRFIYNFYLAHNKELYNNGEKFMSSNRFRVWLNNEYLSEHPEYSWIKEAYSKAVTQSVNNGQTAFTRFFNHESAFPKFKKKGRSDVKMYFVKNNPKDCRCERHRINIPSLGWVRIKEKGYIPTTKDGYVVKSGTVSMKADRYYVSVLVEISDNKIADNSNAGIGIDLGLKDFAIVSNGKTYKNINKSARLKKLEKQFIREQRCLSRKYENLKKGEVTQRANIQKQKLKVQKLHHKIDNIRTDYINKTIAEIVKTKPSYITIEDLNVNGMMKNRHLSKAVASQKFYEFRTKLQIKCNENGIELRIVDRWYPSSKTCHCCGAIKKDLKLSDRIFKCSCGYVEDRDLNAALNLRDAITYEVA

SEQ ID NO: 41 - protein, 392 aa, Ruminococcus sp.
MLTTKKVRLKLTPEQEIQFRKSCGVARWAYNYLLSEKQRVYDEYISNGKTGKKTISEGEVRKYINNVLKPTTHQWLKEVGSNVMKQAVKDADNAYKNFFNGLSKRPKFKSKKSSKQSFYVNYESLTRINGGFKGEKLGFVKTSEPLPKLADGEKYANPRITFDGKYWYLSVVYNIEPKSVQLTNESLGIDLGVKNLAICSNGVTYKNINKSKRVKALKRTLKREQRKLSRKIECNIIGYANNRKPIFRTPLQGCKNIQKQIHYIKLINRKINSIRNNHLHQATAEIVKTKPFQIVMETLNITGMMKNKHLAKAIAEEKLFEFKRQIKYKAEMYGIKVVEVPTFYPSSKTCSVCGCINTNLKLSDRVYHCDSCGITLDRDLNAAINLANYKVI

SEQ ID NO: 42 - protein, 386 aa, Firmicutes bacterium
MRKLLKSFKTEINPTVEQKIKINKTIGTCRYVYNFYLGHNKALYDKGEKFMTGKSFSVWLNNEYVPDNPDKIWIKEAYSKAVKKSIEDGCTAFTRFFKHQSAFPNFKRKGKSDVKMYFVKNNPKDCRCERHRLNIPTLGWVRMKEKGYIPTTKDGWKIKSGTVSIKADRYYVSVLVEIPDAKIANNSNDGIGIDLGLKDLAIVSNGKTYKNINKSARVKKLEKKLRREQRGLSRKYENSKKGESTQKNIQKQKLKVQRLHHKIDNIRTDYINKSIAEIVKTKPSYITIEDLNVSGMMKNRHLSKAVASQKFYEFRTKLKAKCDENGIELRVVDRWYPSSKVCHCCGAIKKDLKLSDRIYRCDCGYVEDRDFNAALNLRDALTYEVA

SEQ ID NO: 43 - protein, 387 aa, Firmicutes bacterium
MWKLLKSFKTEINPSEEQKVKIHKTIGTCRFIYNFYLAHNKELYDNGEKFMSSNKFRVWLNHEYLSEHPEYSWIKEVYSKAVTQAVNNGQTAFARFFNHESAFPNFKKKGKSDVKMYFVKNNPKDCRCERHRINIPSLGWVRIKEKGYIPTTKDGYVIKSGTVSMKADRYYVSVLVEILNNKIANNSNAGIGIDLGLKDFAIVSNGKTYKNINKSARLKKLEKQLIREQRSLSRKYENLKKRESTQKTNIQKQRLKVQKLHHRIDNIRTDYINKTIAEIVKTKPSYITIEDLNVKGMMKNRHLSKAVASQKFYEFKTKLQTKCNENGIELRVVDRWYPSSKTCHCCGAVKKDLKLSDRMFKCSCGYVEDRDFNAALNLRDAITYEVA

SEQ ID NO: 44 - protein, 402 aa, Monoglobales sp.; identical to SEQ ID NO: 29

SEQ ID NO: 45 - protein, 380 aa, Eisenbergiella sp.
MLIPNNVQKTKLFQYAGASRFAYNWALAREKETYEKGGKFISDSELRKEFTRLRHSEEYAWLLNISNNVTKQAIKDACTAYQNFFKGLQKFPRFKSRKRSMPKFYQDNVKIQFSNTHVKFEGFSSSRKANKQKRNWVRLAEHGRIPTDVKYRNPRISFDGLNWWISVCVEFPDSKETLNEDGVGIDLGIKDLAVCSDAVKYKNINKSQKVKKLEKQKRRLQRSISRSYEKNKKGESYCKTNNVIKKEKLLLKRNHRLTNIRKNYLNQTISEIVNRKPRFICIEDLNVRGMMKNRHLSKAVQEQGFFLFRKQLEYKCSDKGVQLIVADRFYPSSKLCSCCGNIKKDLKLSDRVYRCECGNRIDRDFQASINLKAYGEQVAS

SEQ ID NO: 46 - protein, 337 aa, Anaerostipes hadrus
MSSNQFRVWLNNEYISKHPECFWIKEAYSKAVTQAVNNGQAAFTRFFKHQSSFPRFKKKNRSDVKMYFVKNNPKDCRCQRHRINIPSLGWVRIKEKGYIPTTKDGYVIKSGHVSIKAGRYYVSALVEIPNNKIANSSNEGIGVDLGIKDFAVVSNGKVYKNINRSARLKKLEKQLIREQRSLSRRYENLKKGESTQKANIQKQRLKVQKLHHRIDNIRTDHINKTIAEIVKTKPSYITIEDLNISGMMKNRYLSKAVASQKFYEFRIKLQAKCNENGIELRVVDRWYPSSKTCHCCGAIKKDLKLSDRIFKCDCGYTEDRDLNAALNLRDAMTYEVA

SEQ ID NO: 47 - protein, 383 aa, Eisenbergiella sp.
MLKSFKTEIDPTPEQKVKINKTIGTCRYVYNVYLSHNKALYDKGEKFMTGKSFSVWLNNEYIPNNPDKAWIKEVSSKAIKKSIEDGCTAFRRFFKHQSSFPSCKKKGRSDVKMYFVKNNPKDCKCERHRISIPTLGWMRMKEKGYIPTTKDGYAIKSGTVSMKAGRYYVSALVEVPNVNVRNNTNDGVGIDLGLKDLAIVSNGKIYKNINKSARLKKFEKRLRREQRCLSRKYDNRKKGESTQKNIQKQRLKVQRLHHKIENIRTDHINKTIAEIVKTKPSYITIEDLNVSGMMKNRHLSKAVASQKFYEFKIKLKAKCEDNGIELRVVDRFYPSSKLCHCCGRIKKDLKLSDRIYKCECGYIEDRDYNAALNLRDAVTYEVA

SEQ ID NO: 48 - protein, 336 aa, Mageeibacillus indolicus
MTGKSFSVWLNNEYIPNNPEKVWIKEAYSKAVKKSIEDGYTAFTRFFKHQSAFPNFKKKGKSDVKMYFVKNNPKDCRCERHRLNIPTLGWVRIKEKGYIPTTKDGWKIKSGTLSIKAGKYYVSVLVEIPDAKIANNSNDGIGIDLGLKDLAVVSNGKTYKNINKSARVKKLEKKLRREQRCLSRKYENIKEGESTQKNIQKQKLKVQRLHHKIDNIRTDYINKSIAKIVKTKPSYITIEDLNVSGMMKNRHLSKAVASQKFYEFRTKLKAKCDENGIELRVVDRWYPSSKICHCCGAIKKDLKLSDRIYRCDCGYIEDRDLNAALNLRDASTYEIA

SEQ ID NO: 49 - protein, 383 aa, Eubacterium rectale
MLKSFKTEISPTIEQKIKINKTIGTCRYVYNFYLDHNKTLYDNGEKFMTGKSFSVWLNNEYIPNNPDKIWIKEAYSKAVKKSIEDGCTAFTRFFKHQSAFPNFKKKGKSDVKMYFVKNNTKDCRCERHRLNIPTLGWVRIKEKGYIPTTKDGWKIKSGTVSVKADRYYVSVLVEIPDVKIANNSNGGIGIDLGLKDLAIVSNGKTYKNINKSTRIKKLEKKLRREQRCLSRKYENLKKGESTQKNIQKQKLKVQRLHHKIDNIRTDYINKSIAEIVKTKPSYITIENLNVSGMMKNRHLSKAVASQKFYEFRTKLKAKCDENGIELRVVDRWYPSSKICHCCGAIKKDLKLSDRIYHCDCGYVEDRDFNAALNLKDALTYEVA

SEQ ID NO: 50 - protein, 383 aa, Erysipelotrichaceae bacterium SG0102
MLKSFRTEIHPTPEQKVKINKIIGTCRYIYNFYLSNNKALHDQGEAFMSGKAFSVWLNNEYIPDNPDKAWIKEVYSKAVKKSIEDGCLAFTRFFKHQSGFPKFKKKGKSDVKMYFVKNNPKDCICERHRIKIPALGWVRLKEKGYIPTTKDGWKIKSGTVSMKADRYYVSVVVEIPDTKPFCDSGEGIGIDLGLKDFAIVSNGKTYKNINKSAKLKKLEKQLRRAQRCLSRKYENLKKGESTQKNIQKQRLKVQKLYQRIDNIRTDYMNKTIAEIVKTKPSYITIEDLNVKGMMKNRHLSKAVASQKFYEFRTKLKNKCDENGIELRVVDRWYPSSKLCHCCGAIKKDLKLSDRIYKCNCGYIADRDYNASLNLRDAKTYKIA

SEQ ID NO: 51 - protein, 384 aa, Dorea formicigenerans
MLKSFKTEINPTEEQKVKIRKTIGTCRYIYNFYLAHNKELYDKGEKFMSGKSFSVWLNNEYLPQNPDKLWIKEVSSKSVKRSIENGCIAFTRFFKHQSAFPNFKKKGKSDVKMYFVKNNPKDCRCERHRINIPSLGWVRIKEKGYILTTKDGYAIKSGHVSIKADRYYVSVLVEIPNNKIANNSNEGIGIDLGLKDFAIVSNGKTYKNINKSAKLKKLEKQLIKEQRSLSRKYENLKKGESTQKTNIQKQRLKVQKLHHRIDNIRTDYINKTIAEIVKTKPSYITIEDLNISGMMKNKHLSKAVASQKFYEFRIKLQAKCKENGIELRVVDRWFPSSKTCHCCGAVKKDLKLSDRIFKCSCGYVEDRDFNAALNLRDAATYEVA

SEQ ID NO: 52 - protein, 384 aa, Agathobacter rectalis
MLRSFKTEINPSEEQKVKIHKTIGTCRFIYNFYLAHNKELYDNGEKFMSSNRFRVWLNNEYLSEHPEYLWIKEAYSKAVTQSVNNGQTAFTRFFNHESAFPKFKKKGRSDVKMYFVKNNPKDCRCERHRINIPSLGWVRIKEKGYIPTTKDGYVIKSGTVSIKADRYYVSVLVELPDNKTADNSNEGIGIDLGLKDFATVSNGKTYKNINKSAKLKKLEKQLIREQRSLSRKYENLQKGESTQRANIQKQKLKVQKLHHRIDNIRTDYINKTIAEIVKTKPSYITIEDLNVKGMMKNRHLSKAVASQKFYEFRIKLQAKCTENGIELRVADRWYPSSKTCHCCKNIRKDLKLSDRIFKCDCGYIEDRDLNAALNLRDAMTYKVA

SEQ ID NO: 53 - protein, 387 aa, Dorea sp.; identical to SEQ ID NO: 28

SEQ ID NO: 54 - protein, 384 aa, Hungatella sp.
MLKSFKTEINPTEEQKVKIRKTIGTCRYIYNFYLAHNKELHDNGEKFMSGKSFSVWLNNEYLPKNPDKLWIKEVSSKSVKRSIENGCVAFTRFFKHQSAFPNFKKKGKSDVKMYFVKNNPKDCRCERHRMNIPSLGWVRMKEKGYVPTTKDGYVIKSGHVSIKADRYYVSVLIEIPNSKTADNSNEGIGIDLGLKDFAIVSNGKTYKNINKSAKLKKLEKQLIREQRSLSRKYENLKEGESTQRANIQKQKLKVQKVHHKIDDIRTDYINKTIAEMVKTKPSYITIEDLNVSGMMKNKHLSKAVASQKFYEFRTKLQAKCKENGIELRVVDRWYPSSKTCHCCGAIRKDLKLSDRIFECDCGYIEDRDFNAALNLRDATTYEVA

SEQ ID NO: 55 - protein, 384 aa, Agathobacter faecis
MLKSFKTEINPTEEQKVKIRKTIGTCRYIYNFYLAHNKELHDNGEKFMSGKSFSVWLNNEYLPKNPDKLWIKEVSSKSVKRSIENGCVAFTRFFKHQSAFPNFKKKGKSDVKMYFVKNNPKDCRCERHRMNIPSLGWVRMKEKGYVPTTKDGYVIKSGHVSIKADRYYVSVLIEIPNNKIANHSKEGIGIDLGLKDFAIVSNGKTYKNINKSAKLKKLEKQLIREQRSLSRKYENLKKGESTQRANIQKQKLKVQKLHHKIDDIRTDYINKTIAEMVKTKPSYITIEDLNVSGMMKNKHLSKAVASQKFYEFRTKLQAKCKESGIELRVVDRWYPSSKTCHCCGAIKKNLKLSDRIFQCDCGYIEDRDFNAALNLRDATTYEVA

SEQ ID NO: 56 - protein, 384 aa, Clostridium sp.
MLKSFKTEINPTEEQKVKIRKTIGTCRYIYNFYLAHNKELHDNGEKFKSGKSFSVWLNNEYLPQNPDKLWIKEVSSKSVKHSIENGCVAFTRFFKHQSAFPNFKKKGRSDVKMYFVKNNPKDCRCERHRVNIPSLGWVRIKEKGYIPTTKEGYIIKSGHVSMKAGRYYVSALIEIPDNKTADLSNEGIGIDLGLKDFAIVSNGKTYKNINKSARLKKLEKRLVREQRCLSRKYENLKKGESTQRANIQKQKLKVQKLHHKIDNIRTDYINKTIAEIVKTKPSYITIEDLNVSGMMKNKHLSRAVASQKFYEFRIKLKAKSRENGIELRVADRWYPSSKICHCCGMIKKDLKLSDRIFRCHCGYVEDRDFNAALNLRGVKTYKIA

SEQ ID NO: 57 - protein, 387 aa, Fusicatenibacter saccharivorans
MRTLLKSFKTEINPTEEQKVKIRKTIGTCRYIYNFYLAHNKELHENGKKFMSGKRFSVWLNNEYLPKNPDKLWIKEVSSKSVKRSIENGCVAFTRFFKHQSDFPNFKKKGKSNVKMYFVKNNPKDCRCERHRINIPSLGWVRIKEKGYVPTTKDGYVIKSGHVSIKADRYYVSVLVELPDNKTADNSNEGIGIDLGLKDFAIVSNGKTYKNINKSTKLKKLEKQLIREQRSLSRKYENLKKGESTQRANIQKQKLKVQKLHHKIDNIRTDYINKTIAEIVKTKPSYITIEDLNVSGMMKNKHLSRAVASQKFYEFRIKLKAKSRENGIELRVADRWYPSSKICHCCGMIKKDLKLSDRIFRCHCGYVEDRDFNAALNLRGVKTYKIA

SEQ ID NO: 58 - RNA, 185 nt, synthetic construct
  source 1..185: mol_type = other RNA
atgaacgcaaacgtaagtatgtaccgaaggctatttcgggaatttacgactatggagtgcactagaacttgtgagtagatatgatttcggtcaatccaaagcatgcacagtgacatagtaagtaatgttcgtgagaacttacattatctcgatgtgagtatatttaatcacattttgagtggcag

SEQ ID NO: 59 - RNA, 207 nt, synthetic construct
  source 1..207: mol_type = other RNA
ttcacgttttcacgtcttgatacatgtaccgatggctagtcgggaacaggccgttgccttgtgaggcaaggaatacggccaacgcctttggagtgtacaagaacttgtgagtagtctcaggcttgcctggacaaaagcatacacgatgaataaggaatttttctaggcatagataatttctatgttattctatgtttttagtagcag

SEQ ID NO: 60 - RNA, 184 nt, synthetic construct
  source 1..184: mol_type = other RNA
gaaacgcagagatacatatgtaccgaaggccatttcgggaattaacgactgtggagtgtaccagaacttgtgagtagatacagctccggctggtcaaaagcatacacgtttgaaacagtaagtaggattcgtgagaactacaatatctcgatatgagtatatttgatcatattttgagtggcag

SEQ ID NO: 61 - RNA, 184 nt, synthetic construct
  source 1..184: mol_type = other RNA
tcccgcaaacgtaagtatgtaccgaaggctatttcgggaattaacgactgtggagtgtacttaggatctgtgagtagagataactccggttactcaaaagcatacacaaagaaacagtaagcggtattcgtgagaatccgcattatctcgatgtgagtatgtttaatcacattttgagtggcag

SEQ ID NO: 62 - RNA, 187 nt, synthetic construct
  source 1..187: mol_type = other RNA
tgaaaagcaaatgtaagtatgtaccgaaggctatttcgggaattaacgactgtggagtatacaagaacttgtgagtagcatatctgtttacagattgtaaaagcatatacgatgaagcagtaagtaatgttcgtgagaacttacaacatctcgatgtgagtatatttacacacattttgagtggcag

SEQ ID NO: 63 - RNA, 187 nt, synthetic construct
  source 1..187: mol_type = other RNA
ctaaaacgcaaacgtaagtatgtaccgaaggctattttcgggaatttacgactatggagtgtacaagaacttgtgagtagatatgatttcggtcaatccaaagcatacacgatgaaatagtaagtaatgttcgtgagaacttacattatctcgatgtgagcatatttaatcacattttgagtggcag

SEQ ID NO: 64 - RNA, 185 nt, synthetic construct
  source 1..185: mol_type = other RNA
ataaatgcaaacgtaggtatgtaccgaaggctatttcgggaatttacgactatggagtgtacaagaacttgtgagtagatatgatttcggtcaatccaaagcatacacgatgaagtagtaagtagaactcgtgagagtctacattatctcgatgtgagtatgtttaatcacattttgagtagcag

SEQ ID NO: 65 - RNA, 187 nt, synthetic construct
  source 1..187: mol_type = other RNA
ctaaaacgcaaacgtaagtatgtaccgaaggctattttcgggaatttacgactatggagtgtacaagaacttgcgagtagatatgatttcggtcaatccaaagcatacacgatgaaatagtaagtaatgttcgtgagaacttacattatctcgatgtgagcatatttaatcacattttgagtggcag

SEQ ID NO: 66 - RNA, 183 nt, synthetic construct
  source 1..183: mol_type = other RNA
aaaagcagatgtaagtatgtaccgaaggctatttcgggaatttacgactgtggagtgtacaagaacctgtgagtagatatgattttggtcaatcaaaagcatacacaaagaagcagtaagtagaactcgtgagagtttacattatctcgatgtgagtataattacacacattttgagtggcag

SEQ ID NO: 67 - RNA, 186 nt, synthetic construct
  source 1..186: mol_type = other RNA
ttaaaacgcaaatgtaagtatgtaccgaaggctatttcgggaatttacgactgtggagtgtacatgaacttgtgagtagatatgactacggtcaatcaaaaacatacacaatgaagcagtaagtaatgttcgtgagaacttacattatctcgatgtgggtatatttaatcacattttgagtggcag

SEQ ID NO: 68 - RNA, 185 nt, synthetic construct
  source 1..185: mol_type = other RNA
aacgcaaacgtaagtatgtactgcgggctatcgcaggaatttacgactgtggagtgtacaagaacttgtgagtagcgtattgtttacaatcgccaaagcatacacaatgaagcagtaagaagtatccgcaaggacttcaatttctcgatgtgtttgagtatatttcaacacattttgagtggcag

SEQ ID NO: 69 - RNA, 185 nt, synthetic construct
  source 1..185: mol_type = other RNA
ataaacgcaaacgtaggtatgtaccgaaggctatttcgggaatttacgactatggagtgtacaagaacttgtgagtagatatgatttcggtcaatccaaagcatacacgatgaaatagtaagtaaaactcgtgagagtttacattatctcgatgtgagtatatttaatcacattttgagtggcag

SEQ ID NO: 70 - RNA, 187 nt, synthetic construct
  source 1..187: mol_type = other RNA
taaacgcaaacgtaagtatgtactgcgggctatcgcaggaatttacgactgtggagtgtacacgaacttgtgagtagcgtattgtttacaatcgccaaagcatacacatcgaagcagtaagaagtatccgcaaggactttaatttctcgatgtgtttgagtatatttgaacacattttgagtggcag

SEQ ID NO: 71 - DNA, 149 bp, synthetic construct
  source 1..149: mol_type = other DNA
atagattgtatatatgtacggtgggctacatcggaatttacgcctgtggagtgtcacagcaaactgtagtagcaagtgattagcgaggcagggcacgtagaagcaggaatactctaagaatatacatttgtctatatttttagtagcag

SEQ ID NO: 72 - RNA, 155 nt, synthetic construct
  source 1..155: mol_type = other RNA
cacctaaaacgttaacgctaatatgtacgattcgttgcatcggaatttacgcctgtggagtgttacaccaaacgaaagtagcttcggcaaaatcggacacgatgaatcaggaagcaaacaagaatttataagtttttataatttcttggcaacgg

SEQ ID NO: 73 - RNA, 168 nt, synthetic construct
  source 1..168: mol_type = other RNA
cactgaaacgttaatgcaaatatgtacggatacgttagtccggaatttacgcctgtggagagtacaagaacttgtgagtagattgatatttatatcatcaaaagcatactcgttgaagcaggaatgaaacatggaagtttataactttttataagttttcagtaacgg

SEQ ID NO: 74 - RNA, 186 nt, synthetic construct
  source 1..186: mol_type = other RNA
ggaagcaaatgtaagtatgtaccgaaggctatttcgggaattaacgactgtggagtgtacatggacctacgagtagatatgatttcggtcaatcaaaagtatacacactgaagcagtaagtaagattcgtgagaacttacattatctcgatgtgataagtatatttaatcacattttgagtggcag

SEQ ID NO: 75 - RNA, 184 nt, synthetic construct
  source 1..184: mol_type = other RNA
tcctgcaaacgtaagtatgtaccgaaggctatttcgggaattaacgactgtggagtgtacttaggatctgtgagtagagataacgcaggttactcaaaaacatacacgaagaaacagtaagcggtattcgcgagaagccgcattatctcaatgtgagtatgtttaatcacattttgagtggcag

SEQ ID NO: 76 - RNA, 186 nt, synthetic construct
  source 1..186: mol_type = other RNA
ttaacgcaacgtaagtatgtaccgaaggctatttcgggaattaacgactgtggagtgtacaagaacttgtgagtagcgtattgcttgcaatcgccaaagcatacacattgaagcagtaagaagtatccgtgaggacttcagtttctcgatgtgtttgagtatatttaaacgcattttgagtggcag

SEQ ID NO: 77 - RNA, 187 nt, synthetic construct
  source 1..187: mol_type = other RNA
tgaacgcaaatgtaagtatgtaccgaaggctatttcgggaattaacgactgtggagtgtaccagaacttgtgagtagtgagttacttgtaaccacaaaagcatacatggtgaagcagtaagaagtatccgtgaggacttcaatttctcgatgtgattgagtatgttcaaacacattttgagtggcag

SEQ ID NO: 78 - RNA, 186 nt, synthetic construct
  source 1..186: mol_type = other RNA
ttaaaacgcaaatgtaagtatgtaccgaaggctatttcgggaatttacgactgtggagtgtacatgaacttgtgagtagatatgactacggtcaatcaaaaacatacacaatgaagcagtaagtaatgttcgcgagaacttacattatctcgatgtgggtatatttaatcacattttgagtggcag

SEQ ID NO: 79 - RNA, 151 nt, synthetic construct
  source 1..151: mol_type = other RNA
aatcaaaagcacttatatatgtacggagggctaacttcggaatttaagcctttggagagccatacaaatcgtagtagcttaggcaaggcgaggctttatgaagaaggaataatctccatatggatatatttgaccatattttgagtagcag

SEQ ID NO: 80 - RNA, 168 nt, synthetic construct
  source 1..168: mol_type = other RNA
cactgaaacgttaatgcaaatatgtacggatacgttagtccggaatttacgcctatggagagtacaagaacttgtgagtagatagatatttatatcatcaaaagcatactcgttgaagtaggaatgaaacatggaagtttataactttttataagttttcagtaacgg

SEQ ID NO: 81 - RNA, 168 nt, synthetic construct
  source 1..168: mol_type = other RNA
cactgaaacgttaatgcaaatatgtacggatacgttagtccggaatttacgcctatggagagtacaagaacttgtgagtagatagatatttatatcatcaaaagcatactcgttgaagtaggaatgaaacatagaagtttgtaactttttataagttttcagtaacgg

SEQ ID NO: 82 - RNA, 168 nt, synthetic construct
  source 1..168: mol_type = other RNA
cactttcaagttaatacagatatgtactgattcgttagtcaggaatttacgcctatggagagtacaagaacttgtaagtagtgattgacttaccaacacgaaagcatactcgttgaaataggaatgaaacataaaagtttataactttttataagttttcagtaacgg

SEQ ID NO: 83 - RNA, 168 nt, synthetic construct
  source 1..168: mol_type = other RNA
cactgaaacgttaatgcaaatatgtacggatacgttagtccggaatttacgcctatggagagtacaagaacttgcgagtagatagatatttatatcatcaaaagcatactcgttgaagtaggaatgaaacatgggagtttataactttttataagttttcagtaacgg

SEQ ID NO: 84 - RNA, 188 nt, synthetic construct
  source 1..188: mol_type = other RNA
ttaaaagcaaatgtaagtatgtaccgaaggctatttcgggaattaacgactgtggagtgtacaagaacctgtgagtagcgtattgcctgcaatcgtcaaaacatacacaatgaagcagtaagaagtattcgtgaggacttcaatttctcgatgtgtttgagtatatttaaacatatttggagtggcag

SEQ ID NO: 85 - RNA, 185 nt, synthetic construct
  source 1..185: mol_type = other RNA
ataaacgcaaacgtaggtatgtaccgaaggctatttcgggaatttacgactatggagtgtacaagaacttgtgagtagatatgatttcggtcaatccaaagcatacacgatgaaatagtaagtaatgttcgtgagaacttacattatctcgatgtgagtatatttaatcatattttgagtggcag

SEQ ID NO: 86 - RNA, 138 nt, synthetic construct
  source 1..138: mol_type = other RNA
tacgttagtcaggaatttatgcctatggagtgtacaagaacttgcgagtagattatgagaaatcatgtcaaaagcatatacgatgaagtaggaatgaaacataaaggtttataactttttataagttttcagtaacgg

SEQ ID NO: 87 - RNA, 168 nt, synthetic construct
  source 1..168: mol_type = other RNA
gattgaaacgttaatgcaaatatgtacggatacgttagtccggaatttacgcctatggagagtacaagaacttgtgagtagatagatatttatatcgtcaaaagcatactcgttgaagtaggaatgaaacatagaagtttataactttttataagttttcagtaacgg

SEQ ID NO: 88 - RNA, 168 nt, synthetic construct
  source 1..168: mol_type = other RNA
cacttaaatgttaatgcaaatatgtacggatgcgttaattcggaatttacgcctatggagagtacaagaacttgtgagtagataggtatttatgccatcaaaagcatactcgttgaagtaggaatgaaacataaaagtttataactttttataagttttcagtaacgg

SEQ ID NO: 89 - RNA, 168 nt, synthetic construct
  source 1..168: mol_type = other RNA
cactgaaacgttaatgcaaatatgtacggatacgttagtccggaatttacgcctacggagagtacaagaacttgtgagtagatagatatttatatcatcaaaagcatactcgttgaagtaggaatgaaacatagaagtttataactttttataagttttcagtaacgg

SEQ ID NO: 90 - RNA, 155 nt, synthetic construct
  source 1..155: mol_type = other RNA
tttcacaaacaagaaaatgctaatgtgtaggattcgttgtatccgaatttaagcctttggagagttatattaaacgaaagtagctacggcaaaatcggattctatgaagaaggaaataaacaaatttctatatttttatagatttttggcaacgg

SEQ ID NO: 91 - RNA, 155 nt, synthetic construct
  source 1..155: mol_type = other RNA
tttcacaagcaagaaaatgctaatatgtaggattcgttgtatccgaatttaagcctttggagaatcatatcaaacgaaagtagctacggcaaaatcggattcaataaagaaggaaataaacaaatttttatatttttatagatttttggcaacgg

SEQ ID NO: 92 - RNA, 196 nt, synthetic construct
  source 1..196: mol_type = other RNA
tagagaagttctgatatatgtaccgatggctagtcgggaacaggctcttatccttgcattgcaaggagcgtgaagccaacgccttcggagtgttatacaaacgtcagtagcctgtctttcggacggcgagggcgaacacgatgaacaaggaatatttctaagatacatacattgagggttatgttcttagtagcag

SEQ ID NO: 93 - RNA, 200 nt, synthetic construct
  source 1..200: mol_type = other RNA
ttcacgctctcacatttgataaatgtaccgatggctagtcggaaacaggctgttgccttgcctagcaaggaatacagccaacgcctttggagtgtacaagaacttgtgagtagtctcaggcttgcctgggcaaaagcatacacgatgaataaggaatttttctaagacatgcacatttttgtctatgtttttagtagcag

SEQ ID NO: 94 - RNA, 219 nt, synthetic construct
  source 1..219: mol_type = other RNA
aaagaagtccatgcagatatgtaccgattcgttagtcgggaacagacgtgccttcttgcgatggtaaggagtgtcatgtcaaagcctccggagcattatatcaaacgtgagtagcttgtccttcgggatggcaaaaacgaatgcgatgaacgaggaatgaaacgtaaaagtcagtttttcatcaatagactatggctttttataagttttcagtaacgg

SEQ ID NO: 95 - RNA, 172 nt, synthetic construct
  source 1..172: mol_type = other RNA
actgtaaactaaatgtgtaccgatacgttagtcgggaatttaagcctttggagaagtatacaaactatagtagctattctttgaatggtgaaataggctttggtgaattaggaaatagagtttgtagttttttataagtaatttatagaaatttatagattttatgtaacgg

SEQ ID NO: 96 - RNA, 168 nt, synthetic construct
  source 1..168: mol_type = other RNA
cactaaaacgttagtgcaaatatgtacgggtacgttaattcggaatttacgcctatggagagtacaagaacttgtgagtagatagatatttatatcatcaaaagcatactcgttgaagtaggaatgaaacatagaagtttataactttttataagttttcagtaacgg

SEQ ID NO: 97 - DNA, 187 bp, synthetic construct
  source 1..187: mol_type = other DNA
ctaaaacgcaaacgtaagtatgtaccgaaggctattttcgggaatttacgactgcggagtgtacaagaacttgtgagtagatatgatttcggtcaatcaaaaacatacacggtgaagcagtaagtagaactcgtgagagtctacgttatctcgatgtgagtatatttacacatattttgagtggcag

SEQ ID NO: 98 - RNA, 189 nt, synthetic construct
  source 1..189: mol_type = other RNA
ttcactataaagaattttataactatgtacctatcgttactggggaatttaagtctacagagtgttataacaaatgagagtagcttaggcaaaatcagacacgatgaagtagaaagtctaattcgtgagaatagacatggtgtagatatttataaattataatagatttgtacatatttatcgtaacgg

SEQ ID NO: 99 - RNA, 187 nt, synthetic construct
  source 1..187: mol_type = other RNA
tgaacgcaaacgtaagtatgtactgcgggctatcgcaggaatttacgactgtggagtgtacaagaacttgtgagtagcgtattgtttacaatcgccaaagcatacacaatgaagcagtaagaagtatccgcaaggacttcaatttctccatgtgtttgagtatatttaaacatattttgagtggcag

SEQ ID NO: 100 - RNA, 187 nt, synthetic construct; identical to SEQ ID NO: 65
  source 1..187: mol_type = other RNA

SEQ ID NO: 101 - RNA, 138 nt, synthetic construct; identical to SEQ ID NO: 86
  source 1..138: mol_type = other RNA

SEQ ID NO: 102 - RNA, 168 nt, synthetic construct
  source 1..168: mol_type = other RNA
gactgaaacgttaatgcaaatatgtacggatacgttagtccggaatttacgcctatggagagtacaagaacttgtgagtagatagatatttatatcatcaaaagcatactcgttgaagtaggaatgaaacataaaagtttataactttttataagttttcagtaacgg

SEQ ID NO: 103 - RNA, 185 nt, synthetic construct
  source 1..185: mol_type = other RNA
ataaacgcaaacgtaggtatgtaccgaaggctatttcgggaatttacgactatggagtgtacaagaacttgtgagtagatatgatttcggtcaatccaaagcatacacgatgaagtagtaagtagaactcgtgagagtctacgttatctcgatgtgagtatatttacacatattttgagtggcag

SEQ ID NO: 104 - RNA, 195 nt, synthetic construct
  source 1..195: mol_type = other RNA
ataaacgcaaacataagtatgtaccgaaggctatttcgggaattaacgactgtggagtgtacaagaacttgtgagtagcgtattttttatttcttgcaatcgccaaaacatacacaatgaagcagtaagaagaatccgtgaggacttcaatttctcgatgtgtttgtgtatatttaatcacattttgagtggcag

SEQ ID NO: 105 - RNA, 188 nt, synthetic construct
  source 1..188: mol_type = other RNA
tgaaagcaaacgtaagtatgtactgcgggctatcgcaggaatttacgactgtggagtgtacaagaacttgtgagtagcgaattgtttacaatcgccaaagcatacacattgaagcagtaagaagtatccgcaaggacttcaatttctcgatgcgtttgagtatatttcaacacattttgagtggcaga

SEQ ID NO: 106 - RNA, 188 nt, synthetic construct
  source 1..188: mol_type = other RNA
tcaacgcaaacgtaagtatgtactgcgggctatcgcaggaatttacgactgtggagtgtacaagaacttgtgagtagcgtattgtttacaatcgccaaagcatacacaatgaagcagtaagaagtatccgcaaggactttaatttctcgatgtgtttgagaatatttaaacacattttgagtggcaga

SEQ ID NO: 107 - RNA, 187 nt, synthetic construct
  source 1..187: mol_type = other RNA
acaagcaaatgtaagtatgtaccgatggcttagtcgggaatttacgactgtggagtgtacaagaacttgtgagtagtatgtcacttgtgactacaaaagcatacacgaagaagcagtaagtaatgttcgtgagaacttacatatctcgatgtgtttgagtatatttaaacacattttgagtagcaga

SEQ ID NO: 108 - RNA, 186 nt, synthetic construct
  source 1..186: mol_type = other RNA
ataaaacgcaaacgtaggtatgtaccgaaggctgtttcgggaatttacgactatggagtgtacaagaacttgtgagtagatatgatttcggtcaatccaaagcatacacgatgaagtagtaagtagaactcgtgagagtctacgttatctcgatgtgagtatatttaatcacattttgagtggcag

SEQ ID NO: 109 - RNA, 185 nt, synthetic construct
  source 1..185: mol_type = other RNA
ataaacgcaaacgtaggtatgtaccgaaggctatttcgggaatttacgactgtggagtgtacaagaacttgtgagtagatatgatttcggtcaatccaaagcatacacgataaagcagtaagtagaactcgtgagggtctacattatctcgatgtgagtatatttaatcacattttgagtggcag

SEQ ID NO: 110 - RNA, 185 nt, synthetic construct; identical to SEQ ID NO: 85
  source 1..185: mol_type = other RNA

SEQ ID NO: 111 - RNA, 185 nt, synthetic construct
  source 1..185: mol_type = other RNA
ataaacgcaaacgtaggtatgtaccgtgggcttacacgggaattaacgactgtggagtgtacaagaacttgtgagtagatatgattttggtcaatccaaagcatacacgatgaaacagtaagtaaaacttgtgagagtttacattatctcgatgtgagtatatttacacacattttgagtggcag

SEQ ID NO: 112 - RNA, 185 nt, synthetic construct
  source 1..185: mol_type = other RNA
ataaacgcaaacgtaggtatgtaccgtgggcttacacgggaattaacgactgtggagtgtacaagaacttgtgagtagatatgattttggtcaatccaaagcatacacgatgaaacagtaagtaaaacttgtgagagtttacattatctcgatgtgagtatatttacatacattttgagtggcag

SEQ ID NO: 113 - RNA, 186 nt, synthetic construct
  source 1..186: mol_type = other RNA
ggacgcaaatgtaagtatgtaccgaaggctatttcgggaattaacgactgtggagtgtacatggatctacgagtagatatgatttcggtcaatcaaaagtatacacaaggaagcagtaagtaagattcgtgagaacttacattatctcgatgtgataagtatatttaatcacattttgagtggcag

SEQ ID NO: 114 - RNA, 186 nt, synthetic construct; identical to SEQ ID NO: 113
  source 1..186: mol_type = other RNA

SEQ ID NO: 115 - DNA, 1464 bp, synthetic construct
  source 1..1464: mol_type = other DNA
atgaggaaattgctgaagagcttcaagacggaaataaatccaacagaagagcagaaagtcaggattcgtaaaacaataggtacttgcagatttatctataacttctatcttgctcataataaggagcttcatgaaagtggcaaaaagtttatgagcagcagccaattcagagtatggctcaacaatgaatatcttccgagccatccggaatattcctggatcaaggaagcttattcaaaatcggtaacacaggcagtaaatgatggacagaccgcatttacaagattctttaatcacaagagcgcctttccaaagtttaaaaagaaaggcaagtctgatgtgaaaatgtattttgtaaggaataatccaaaagattgcagctgcgaaagacacagaatcaagattccttcacttggctgggtccgtatcaaagagaaaggatatattcccactacaaaagatggatatgtaattaagagcggtcatgtctcaataaaagctgatagatactatgtttcagttcttatagaaatcccagacaaaacgtcagctagtaattccagtgaaggaattggcattgaccttggattaaaggactttgcgattgcttctaatggaaagacttataagaacatcaacaaatctgctaaattaaagaagcttgaaaaaaagcttattcgagaacagagaagtctttctcgaaagtatgaaaatataaagaaaggagggtccactcaaaaaagaaatatacaaaaacaaaggcttaagatacagaaacttcatcatagaatcgacaatattcgtactgattacatcaataagataatcgcagagatagtgaaaaccaagccatcttatataacgattgaagatctaaacatatcagggatgatgaagaacagacatctttcaaaggcagttgcttcgcagaagttttatgaatttaagacaaagcttcaagctaaatgcagggagaacggaatcgaacttcgagttgtagatagatggttcccatcatctaagacttgtcactgctgtaaaagtatcaagaaagatttaaagctttcagatagacttttcagatgtgattgtggatatatcgaagacagagatttcaatgctgcactaaatctgagagatgctacaacttacgaagttgcaagcagccatcaccatcatcaccactaaatgaacgcaaacgtaagtatgtaccgaaggctatttcgggaatttacgactatggagtgcactagaacttgtgagtagatatgatttcggtcaatccaaagcatgcacagtgacatagtaagtaatgttcgtgagaacttacattatctcgatgtgagtatatttaatcacattttgagtggcagctgatggtccatgtctgttaggccggcatggtcccagcctcctcgctggcgccggctgggcaacatgcttcggcatggcgaatgggacccg

SEQ ID NO: 116 - DNA, 20 bp, synthetic construct
  source 1..20: mol_type = other DNA
ctgatggtccatgtctgtta

SEQ ID NO: 117 - DNA, 1463 bp, synthetic construct
  source 1..1463: mol_type = other DNA
atgaggaaattgctgaagagcttcaagacggaaataaatccaacagaagagcagaaagtcaggattcgtaaaacaataggtacttgcagatttatctataacttctatcttgctcataataaggagcttcatgaaagtggcaaaaagtttatgagcagcagccaattcagagtatggctcaacaatgaatatcttccgagccatccggaatattcctggatcaaggaagcttattcaaaatcggtaacacaggcagtaaatgatggacagaccgcatttacaagattctttaatcacaagagcgcctttccaaagtttaaaaagaaaggcaagtctgatgtgaaaatgtattttgtaaggaataatccaaaagattgcagctgcgaaagacacagaatcaagattccttcacttggctgggtccgtatcaaagagaaaggatatattcccactacaaaagatggatatgtaattaagagcggtcatgtctcaataaaagctgatagatactatgtttcagttcttatagaaatcccagacaaaacgtcagctagtaattccagtgaaggaattggcattgaccttggattaaaggactttgcgattgcttctaatggaaagacttataagaacatcaacaaatctgctaaattaaagaagcttgaaaaaaagcttattcgagaacagagaagtctttctcgaaagtatgaaaatataaagaaaggagggtccactcaaaaaagaaatatacaaaaacaaaggcttaagatacagaaacttcatcatagaatcgacaatattcgtactgattacatcaataagataatcgcagagatagtgaaaaccaagccatcttatataacgattgaagatctaaacatatcagggatgatgaagaacagacatctttcaaaggcagttgcttcgcagaagttttatgaatttaagacaaagcttcaagctaaatgcagggagaacggaatcgaacttcgagttgtagatagatggttcccatcatctaagacttgtcactgctgtaaaagtatcaagaaagatttaaagctttcagatagacttttcagatgtgattgtggatatatcgaagacagagatttcaatgctgcactaaatctgagagatgctacaacttacgaagttgcaagcagccatcaccatcatcaccactaaatgaacgcaaacgtaagtatgtaccgaaggctatttcgggaatttacgactatggagtgcactagaacttgtgagtagatatgatttcggtcaatccaaagcatgcacagtgacatagtaagtaatgttcgtgagaacttacattatctcgatgtgagtatatttaatcacattttgagtggcagctgatggtccatgtctgttaggccggcatggtcccagcctcctcgctggcgccggctgggcaacatgcttcggcatggcgaatgggaccc

SEQ ID NO: 118 - DNA, 2754 bp, synthetic construct
  source 1..2754: mol_type = other DNA
gcgcccaatacgcaaaccgcctctccccgcgcgttggccgattcattaatgcagctggcacgacaggtttcccgactggaaagcgggcagtgagcgcaacgcaattaatgtgagttagctcactcattaggcaccccaggctttacactttatgcttccggctcgtatgttgtgtggaattgtgagcggataacaatttcacacaggaaacagctatgaccatgattacgccaagcttgcatgcctgcaggcctggacatccgcgagcacagctaaggccannnnnnnctgatggtccatgtctgttactcacaccgaccggcacagcatcaagaagcgggtaccgagctcgaattcactggccgtcgttttacaacgtcgtgactgggaaaaccctggcgttacccaacttaatcgccttgcagcacatccccctttcgccagctggcgtaatagcgaagaggcccgcaccgatcgcccttcccaacagttgcgcagcctgaatggcgaatggcgcctgatgcggtattttctccttacgcatctgtgcggtatttcacaccgcatatggtgcactctcagtacaatctgctctgatgccgcatagttaagccagccccgacacccgccaacacccgctgacgcgccctgacgggcttgtctgctcccggcatccgcttacagacaagctgtgaccgtctccgggagctgcatgtgtcagaggttttcaccgtcatcaccgaaacgcgcgagacgaaagggcctcgtgatacgcctatttttataggttaatgtcatgataataatggtttcttagacgtcaggtggcacttttcggggaaatgtgcgcggaacccctatttgtttatttttctaaatacattcaaatatgtatccgctcatgagacaataaccctgataaatgcttcaataatattgaaaaaggaagagtatgagtattcaacatttccgtgtcgcccttattcccttttttgcggcattttgccttcctgtttttgctcacccagaaacgctggtgaaagtaaaagatgctgaagatcagttgggtgcacgagtgggttacatcgaactggatctcaacagcggtaagatccttgagagttttcgccccgaagaacgttttccaatgatgagcacttttaaagttctgctatgtggcgcggtattatcccgtattgacgccgggcaagagcaactcggtcgccgcatacactattctcagaatgacttggttgagtactcaccagtcacagaaaagcatcttacggatggcatgacagtaagagaattatgcagtgctgccataaccatgagtgataacactgcggccaacttacttctgacaacgatcggaggaccgaaggagctaaccgcttttttgcacaacatgggggatcatgtaactcgccttgatcgttgggaaccggagctgaatgaagccataccaaacgacgagcgtgacaccacgatgcctgtagcaatggcaacaacgttgcgcaaactattaactggcgaactacttactctagcttcccggcaacaattaatagactggatggaggcggataaagttgcaggaccacttctgcgctcggcccttccggctggctggtttattgctgataaatctggagccggtgagcgtgggtctcgcggtatcattgcagcactggggccagatggtaagccctcccgtatcgtagttatctacacgacggggagtcaggcaactatggatgaacgaaatagacagatcgctgagataggtgcctcactgattaagcattggtaactgtcagaccaagtttactcatatatactttagattgatttaaaacttcatttttaatttaaaaggatctaggtgaagatcctttttgataatctcatgaccaaaatcccttaacgtgagttttcgttccactgagcgtcagaccccgtagaaaagatcaaaggatcttcttgagatcctttttttctgcgcgtaatctgctgcttgcaaacaaaaaaaccaccgctaccagcggtggtttgtttgccggatcaagagctaccaactctttttccgaaggtaactggcttcagcagagcgcagataccaaatactgttcttctagtgtagccgtagttaggccaccacttcaagaactctgtagcaccgcctacatacctcgctctgctaatcctgttaccagtggctgctgccagtggcgataagtcgtgtcttaccgggttggactcaagacgatagttaccggataaggcgcagcggtcgggctgaacggggggttcgtgcacacagcccagcttggagcgaacgacctacaccgaactgagatacctacagcgtgagctatgagaaagcgccacgcttcccgaagggagaaaggcggacaggtatccggtaagcggcagggtcggaacaggagagcgcacgagggagcttccagggggaaacgcctggtatctttatagtcctgtcgggtttcgccacctctgacttgagcgtcgatttttgtgatgctcgtcaggggggcggagcctatggaaaaacgccagcaacgcggcctttttacggttcctggccttttgctggccttttgctcacatgttctttcctgcgttatcccctgattctgtggataaccgtattaccgcctttgagtgagctgataccgctcgccgcagccgaacgaccgagcgcagcgagtcagtgagcgaggaagcggaaga

SEQ ID NO: 119 - DNA, 2700 bp, synthetic construct
  source 1..2700: mol_type = other DNA
tgagtgataacactgcggccaacttacttctgacaacgatcggaggaccgaaggagctaaccgcttttttgcacaacatgggggatcatgtaactcgccttgatcgttgggaaccggagctgaatgaagccataccaaacgacgagcgtgacaccacgatgcctgtagcaatggcaacaacgttgcgcaaactattaactggcgaactacttactctagcttcccggcaacaattaatagactggatggaggcggataaagttgcaggaccacttctgcgctcggcccttccggctggctggtttattgctgataaatctggagccggtgagcgtgggtctcgcggtatcattgcagcactggggccagatggtaagccctcccgtatcgtagttatctacacgacggggagtcaggcaactatggatgaacgaaatagacagatcgctgagataggtgcctcactgattaagcattggtaactgtcagaccaagtttactcatatatactttagattgatttaaaacttcatttttaatttaaaaggatctaggtgaagatcctttttgataatctcatgaccaaaatcccttaacgtgagttttcgttccactgagcgtcagaccccgtagaaaagatcaaaggatcttcttgagatcctttttttctgcgcgtaatctgctgcttgcaaacaaaaaaaccaccgctaccagcggtggtttgtttgccggatcaagagctaccaactctttttccgaaggtaactggcttcagcagagcgcagataccaaatactgttcttctagtgtagccgtagttaggccaccacttcaagaactctgtagcaccgcctacatacctcgctctgctaatcctgttaccagtggctgctgccagtggcgataagtcgtgtcttaccgggttggactcaagacgatagttaccggataaggcgcagcggtcgggctgaacggggggttcgtgcacacagcccagcttggagcgaacgacctacaccgaactgagatacctacagcgtgagctatgagaaagcgccacgcttcccgaagggagaaaggcggacaggtatccggtaagcggcagggtcggaacaggagagcgcacgagggagcttccagggggaaacgcctggtatctttatagtcctgtcgggtttcgccacctctgacttgagcgtcgatttttgtgatgctcgtcaggggggcggagcctatggaaaaacgccagcaacgcggcctttttacggttcctggccttttgctggccttttgctcacatgttctttcctgcgttatcccctgattctgtggataaccgtattaccgcctttgagtgagctgataccgctcgccgcagccgaacgaccgagcgcagcgagtcagtgagcgaggaagcggaagagcgcccaatacgcaaaccgcctctccccgcgcgttggccgattcattaatgcagctggcacgacaggtttcccgactggaaagcgggcagtgagcgcaacgcaattaatgtgagttagctcactcattaggcaccccaggctttacactttatgcttccggctcgtatgttgtgtggaattgtgagcggataacaatttcacacaggaaacagctatgaccatgattacgccaagcttgcatgcctgcaggcctggacatccgcgagcacagctaaggccagggaggagctgatggtccatgtctgttactcacaccgaccggcacagcatcaagaagcgggtaccgagctcgaattcactggccgtcgttttacaacgtcgtgactgggaaaaccctggcgttacccaacttaatcgccttgcagcacatccccctttcgccagctggcgtaatagcgaagaggcccgcaccgatcgcccttcccaacagttgcgcagcctgaatggcgaatggcgcctgatgcggtattttctccttacgcatctgtgcggtatttcacaccgcatatggtgcactctcagtacaatctgctctgatgccgcatagttaagccagccccgacacccgccaacacccgctgacgcgccctgacgggcttgtctgctcccggcatccgcttacagacaagctgtgaccgtctccgggagctgcatgtgtcagaggttttcaccgtcatcaccgaaacgcgcgagacgaaagggcctcgtgatacgcctatttttataggttaatgtcatgataataatggtttcttagacgtcaggtggcacttttcggggaaatgtgcgcggaacccctatttgtttatttttctaaatacattcaaatatgtatccgctcatgagacaataaccctgataaatgcttcaataatattgaaaaaggaagagtatgagtattcaacatttccgtgtcgcccttattcccttttttgcggcattttgccttcctgtttttgctcacccagaaacgctggtgaaagtaaaagatgctgaagatcagttgggtgcacgagtgggttacatcgaactggatctcaacagcggtaagatccttgagagttttcgccccgaagaacgttttccaatgatgagcacttttaaagttctgctatgtggcgcggtattatcccgtattgacgccgggcaagagcaactcggtcgccgcatacactattctcagaatgacttggttgagtactcaccagtcacagaa

SEQ ID NO: 120 - DNA, 60 bp, synthetic construct
  source 1..60: mol_type = other DNA
cctggacatccgcgagcacagctaaggccannnnnnnctgatggtccatgtctgttactc

SEQ ID NO: 121 - DNA, 49 bp, synthetic construct
  source 1..49: mol_type = other DNA
cttcttgatgctgtgccggtcggtgtgagtaacagacatggaccatcag

SEQ ID NO: 122 - DNA, 38 bp, synthetic construct
  source 1..38: mol_type = other DNA
ggcacagcatcaagaagcgggtaccgagctcgaattca

SEQ ID NO: 123 - DNA, 43 bp, synthetic construct
  source 1..43: mol_type = other DNA
agctgtgctcgcggatgtccaggcctgcaggcatgcaagcttg

SEQ ID NO: 124 - DNA, 73 bp, synthetic construct
  source 1..73: mol_type = other DNA
ctcctcgctggcgccggctgggcaacatgcttcggcatggcgaatgggacccggaattcccgggtcgactcga

SEQ ID NO: 125 - DNA, 83 bp, synthetic construct
  source 1..83: mol_type = other DNA
ccagccggcgccagcgaggaggctgggaccatgccggcctaacagacatggaccatcagctgccactcaaaatgtgattaaat

SEQ ID NO: 126 - DNA, 27 bp, synthetic construct
  source 1..27: mol_type = other DNA
tgagtgataacactgcggccaacttac

SEQ ID NO: 127 - DNA, 28 bp, synthetic construct
  source 1..28: mol_type = other DNA
ttctgtgactggtgagtactcaaccaag

SEQ ID NO: 128 - DNA, 55 bp, synthetic construct
  source 1..55: mol_type = other DNA
ggccaccattaggagctgatggtccatgtctgttactcacaccgaccggcacagc

SEQ ID NO: 129 - DNA, 55 bp, synthetic construct
  source 1..55: mol_type = other DNA
gctgtgccggtcggtgtgagtaacagacatggaccatcagctcctaatggtggcc

SEQ ID NO: 130 - DNA, 55 bp, synthetic construct
  source 1..55: mol_type = other DNA
ggccaccattttgatctgatggtccatgtctgttactcacaccgaccggcacagc

SEQ ID NO: 131 - DNA, 55 bp, synthetic construct
  source 1..55: mol_type = other DNA
gctgtgccggtcggtgtgagtaacagacatggaccatcagatcaaaatggtggcc

SEQ ID NO: 132 - DNA, 50 bp, synthetic construct
  source 1..50: mol_type = other DNA
cggtatttcacaccgcatatggtgcactctcagtacaatctgctctgatg

SEQ ID NO: 133 - DNA, 20 bp, synthetic construct
  source 1..20: mol_type = other DNA
taacagacatggaccatcag

SEQ ID NO: 134 - DNA, 81 bp, synthetic construct
  source 1..81: mol_type = other DNA
ataaggagctggagaacctggagatcaatctgcggaaggagatcgccaaggccttcaagggcaacgagggctacaagtcct

SEQ ID NO: 135 - DNA, 80 bp, synthetic construct
  source 1..80: mol_type = other DNA
ggacttgtagccctcgttgcccttgaaggccttggcgatctccttccgcagattgatctccaggttctccagctccttat

SEQ ID NO: 136 - DNA, 38 bp, synthetic construct
  source 1..38: mol_type = other DNA
ggagtgagtacggtgtgcataaggagctggagaacctg

SEQ ID NO: 137 - DNA, 42 bp, synthetic construct
  source 1..42: mol_type = other DNA
gagttggatgctggatgggagcggataacaatttcacacagg

SEQ ID NO: 138 - DNA, 3251 bp, synthetic construct
  source 1..3251: mol_type = other DNA
catgttctttcctgcgttatcccctgattctgtggataaccgtattaccgcctttgagtgagctgataccgctcgccgcagccgaacgaccgagcgcagcgagtcagtgagcgaggaagcggaagagcgcctgatgcggtattttctccttacgcatctgtgcggtatttcacaccgcatatgctggatccttgacagctagctcagtcctaggtataatactagtattgtcaccagactggcgtcgttttagagctagaaatagcaagttaaaataaggctagtccgttatcaacttgaaaaagtggcaccgagtcggtgctttttttgaattctctagagtcgacctgcagaagcttagatctattaccctgttatccctactcgagttcatgtgcagctccataagcaaaaggggatgataagtttatcaccaccggggaggagctgatggtccatgtctgttaactatttgcaacagtgccgttgatcgtgctatgatcgactgatgtcatcagcggtggagtgcaatgtcatgagggaagcggtgatcgccgaagtatcgactcaactatcagaggtagttggcgtcatcgagcgccatctcgaaccgacgttgctggccgtacatttgtacggctccgcagtggatggcggcctgaagccacacagtgatattgatttgctggttacggtgaccgtaaggcttgatgaaacaacgcggcgagctttgatcaacgaccttttggaaacttcggcttcccctggagagagcgagattctccgcgctgtagaagtcaccattgttgtgcacgacgacatcattccgtggcgttatccagctaagcgcgaactgcaatttggagaatggcagcgcaatgacattcttgcaggtatcttcgagccagccacgatcgacattgatctggctatcttgctgacaaaagcaagagaacatagcgttgccttggtaggtccagcggcggaggaactctttgatccggttcctgaacaggatctatttgaggcgctaaatgaaaccttaacgctatggaactcgccgcccgactgggctggcgatgagcgaaatgtagtgcttacgttgtcccgcatttggtacagcgcagtaaccggcaaaatcgcgccgaaggatgtcgctgccgactgggcaatggagcgcctgccggcccagtatcagcccgtcatacttgaagctagacaggcttatcttggacaagaagaagatcgcttggcctcgcgcgcagatcagttggaagaatttgtccactacgtgaaaggcgagatcaccaaggtagtcggcaaataagatgccgctcgccagtcgattggctgagctcataagttcctattccgaagttccgcgaacgcgtaaaggatctaggtgaagatcctttttgataatctcatgaccaaaatcccttaacgtgagttttcgttccactgagcgtcagaccccgtagaaaagatcaaaggatcttctcagatccttccgtatttagccagtatgttctctagtgtggttcgttgtttttgcgtgagccatgagaacgaaccattgagatcatacttactttgcatgtcactcaaaaattttgcctcaaaactggtgagctgaatttttgcagttaaagcatcgtgtagtgtttttcttagtccgttatgtaggtaggaatctgatgtaatggttgttggtattttgtcaccattcatttttatctggttgttctcaagttcggttacgagatccatttgtctatctagttcaacttggaaaatcaacgtatcagtcgggcggcctcgcttatcaaccaccaatttcatattgctgtaagtgtttaaatctttacttattggtttcaaaacccattggttaagccttttaaactcatggtagttattttcaagcattaacatgaacttaaattcatcaaggctaatctctatatttgccttgtgagttttcttttgtgttagttcttttaataaccactcataaatcctcatagagtatttgttttcaaaagacttaacatgttccagattatattttatgaatttttttaactggaaaagataaggcaatatctcttcactaaaaactaattctaatttttcgcttgagaacttggcatagtttgtccactggaaaatctcaaagcctttaaccaaaggattcctgatttccacagttctcgtcatcagctctctggttgctttagctaatacaccataagcattttccctactgatgttcatcatctgaacgtattggttataagtgaacgataccgtccgttctttccttgtagggttttcaatcgtggggttgagtagtgccacacagcataaaattagcttggtttcatgctccgttaagtcatagcgactaatcgctagttcatttgctttgaaaacaactaattcagacatacatctcaattggtctaggtgattttaatcactataccaattgagatgggctagtcaatgataattactagtccttttcctttgagttgtgggtatctgtaaattctgctagacctttgctggaaaacttgtaaattctgctagaccctctgtaaattccgctagacctttgtgtgttttttttgtttatattcaagtggttataatttatagaataaagaaagaataaaaaaagataaaaagaatagatcccagccctgtgtataactcactactttagtcagttccgcagtattacaaaaggatgtcgcaaacgctgtttgctcctctacaaaacagaccttaaaaccctaaaggcttaagtagcaccctcgcaagctcggttgcggccgcaatcgggcaaatcgctgaatattccttttgtctccgaccatcaggcacctgagtcgctgtctttttcgtgacattcagttcgctgcgctcacggctctggcagtgaatgggggtaaatggcactacaggcgccttttatggattcatgcaaggaaactacccataatacaagaaaagcccgtcacgggcttctcagggcgttttatggcgggtctgctatgtggtgctatctgactttttgctgttcagcagttcctgccctctgattttccagtctgaccacttcggattatcccgtgacaggtcattcagactggctaatgcacccagtaaggcagcggtatcatcaacaacgccagcaacgcggcctttttacggttcctggccttttgctggccttttgctca

SEQ ID NO: 139 - DNA, 25 bp, synthetic construct
  source 1..25: mol_type = other DNA
aggagctgatggtccatgtctgtta

SEQ ID NO: 140 - DNA, 25 bp, synthetic construct
  source 1..25: mol_type = other DNA
gagggctgatggtccatgtctgtta

SEQ ID NO: 141 - DNA, 25 bp, synthetic construct
  source 1..25: mol_type = other DNA
aggagaggtagggcaaaccgcccct

SEQ ID NO: 142 - DNA, 25 bp, synthetic construct
  source 1..25: mol_type = other DNA
gagggcaaaggcctcccggaagttc

SEQ ID NO: 143 - DNA, 3480 bp, synthetic construct
  source 1..3480: mol_type = other DNA
gagggcctatttcccatgattccttcatatttgcatatacgatacaaggctgttagagagataattggaattaatttgactgtaaacacaaagatattagtacaaaatacgtgacgtagaaagtaataatttcttgggtagtttgcagttttaaaattatgttttaaaatggactatcatatgcttaccgtaacttgaaagtatttcgatttcttggctttatatatcttgtggaaaggacgaaacaccgctaaaacgcaaacgtaagtatgtaccgaaggctattttcgggaatttacgactatggagtgtacaagaacttgtgagtagatatgatttcggtcaatccaaagcatacacgatgaaatagtaagtaatgttcgtgagaacttacattatctcgatgtgagcatatttaatcacattttgagtggcagctgatggtccatgtctgttaggccggcatggtcccagcctcctcgctggcgccggctgggcaacatgcttcggcatggcgaatgggacttttttgttttagagctagaaatagcaagttaaaataaggctagtccgtttttagcgcgtgcgccaattctgcagacaaatggctctagaggtacccgatgtacgggccagatatacgcgttgacattgattattgactagttattaatagtaatcaattacggggtcattagttcatagcccatatatggagttccgcgttacataacttacggtaaatggcccgcctggctgaccgcccaacgacccccgcccattgacgtcaataatgacgtatgttcccatagtaacgccaatagggactttccattgacgtcaatgggtggagtatttacggtaaactgcccacttggcagtacatcaagtgtatcatatgccaagtacgccccctattgacgtcaatgacggtaaatggcccgcctggcattatgcccagtacatgaccttatgggactttcctacttggcagtacatctacgtattagtcatcgctattaccatggtgatgcggttttggcagtacatcaatgggcgtggatagcggtttgactcacggggatttccaagtctccaccccattgacgtcaatgggagtttgttttggcaccaaaatcaacgggactttccaaaatgtcgtaacaactccgccccattgacgcaaatgggcggtaggcgtgtacggtgggaggtctatataagcagagctctctggctaactagagaacccactgcttactggcttatcgaaattaatacgactcactatagggagacccaagctggctagcgtttaaacttaagcttggtaccgagctcggatccgccaccatggactataaggaccacgacggagactacaaggatcatgatattgattacaaagacgatgacgataagatggccccaaagaagaagcggaaggtcggtatccacggagtcccagcagccatgtggaaattgctaaagagcttcaagacggaaataaatccgtcagaggaacagaaagtcaagattcataagacgataggaacttgtagattcatttataatttctatcttgctcataacaaagaactttacgataaaggcgaaaagtttatgagtggtaaaagttttagtgtttggctgaacaatgagtatcttccacaaaatccagacaagttatggattaaggaagtcagttcaaaatctgtaaagcactcaattgaaaatggttgtatcgcatttaccagatttttcaaacatcaaagtgcttttccgaatttaaaaaagaaaggcaaatctgatgtaaaaatgtattttgtaaagaataatccaaaagattgtcgttgcgaaagacacagaatcaatattccgtcacttggttgggttcgcatcaaagaaaaaggatatattccaacaactaaagacggatatgtgattaaaagcggcacggtctcaatgaaagctgacagatactatgtttcagttcttgtagaaatttcaaataacaagatagccaataattccaatgcaggaattggcattgaccttggattaaaggattttgccattgtttctaatggtaaaacttataagaacattaacaaatctgcaagattaaagaaacatgaaaaacagcttattcgagaacagagaagtctttctcgaaagtatgaaaatttaaagaaaggagagtccactcaaaaagcaaatatacaaaaacaaaggcttaaggtacagaaacttcatcatagaatggataatattcgtactgattacatcaataaaacaatcgcagagatagtaaaaaccaaaccatcttatattacgattgaagatttgaatgtaaaaggtatgatgaaaaacagacatctttcaaaagctgttgcttcacagaagttttatgaatttagaacaaagcttcaagctaaatgcaatgaaaatggaatcgaacttcgagtagtagacagatggtatccatcatctaaaacctgtcactgctgtggcgctgtcaaaaaagatttaaagctttcagatagaatatttaaatgcagttgcggttatgtcgaagacagagatttcaatgctgcacttaatttgagagatgcgataacttacgaagttgcaaaaaggccggcggccacgaaaaaggccggccaggcaaaaaagaaaaaggaattcggcagtggagagggcagaggaagtctgctaacatgcggtgacgtcgaggagaatcctggcccagtgagcaagggcgaggagctgttcaccggggtggtgcccatcctggtcgagctggacggcgacgtaaacggccacaagttcagcgtgtccggcgagggcgagggcgatgccacctacggcaagctgaccctgaagttcatctgcaccaccggcaagctgcccgtgccctggcccaccctcgtgaccaccctgacctacggcgtgcagtgcttcagccgctaccccgaccacatgaagcagcacgacttcttcaagtccgccatgcccgaaggctacgtccaggagcgcaccatcttcttcaaggacgacggcaactacaagacccgcgccgaggtgaagttcgagggcgacaccctggtgaaccgcatcgagctgaagggcatcgacttcaaggaggacggcaacatcctggggcacaagctggagtacaactacaacagccacaacgtctatatcatggccgacaagcagaagaacggcatcaaggtgaacttcaagatccgccacaacatcgaggacggcagcgtgcagctcgccgaccactaccagcagaacacccccatcggcgacggccccgtgctgctgcccgacaaccactacctgagcacccagtccgccctgagcaaagaccccaacgagaagcgcgatcacatggtcctgctggagttcgtgaccgccgccgggatcactctcggcatggacgagctgtacaaggaattctaactcgag

SEQ ID NO: 144 - DNA, 25 bp, synthetic construct
  source 1..25: mol_type = other DNA
aggagaaggccaagtggtcccaggc

SEQ ID NO: 145 - DNA, 25 bp, synthetic construct
  source 1..25: mol_type = other DNA
aggagttgtactctggtctgagact

SEQ ID NO: 146 - DNA, 25 bp, synthetic construct
  source 1..25: mol_type = other DNA
aggaggagggcagaatcatcacgaa

SEQ ID NO: 147 - DNA, 25 bp, synthetic construct
  source 1..25: mol_type = other DNA
aggagtctgatgtcgggttatacac

SEQ ID NO: 148 - DNA, 25 bp, synthetic construct
  source 1..25: mol_type = other DNA
aggagacaaagttcctgacattctc

SEQ ID NO: 149 - DNA, 25 bp, synthetic construct
  source 1..25: mol_type = other DNA
aggagaaggccaggtgacagagggt

SEQ ID NO: 150 - protein, 367 aa, NA
MVYKIEISPTQEQKSIIFRTFDATRLVYNYFIEVNKARHENGYPYMGNLEFSKTFNNYMSRLEWVRDKSLKISSKAVKEAMKDADKAYQRFFKGISRYPRFKSRREPRKSYYLCGSIHVKRHAVRLPNLGWVLLKEKNYIPAGSGVVSCRLIYEGGRFYVAILTQDNNSVNNQLSNDGLGVDVGIRFLATDSDKDVYPNINKSSRVKHLKKRLKREQRKLVRRNKKSLRREKTRQIINRIHYKISCICIDHKNKVVSALVKKKPSYITVETLNIKGMLKNRHLSRVIHEQGLHDFMTRLANKARQYGIELRRVSQYFASSKLCSTCGAKNDPKHKTFWVCTSCGTRHDRDINASLNLLNATQYTIDK

SEQ ID NO: 151 - protein, 382 aa, Fusobacterium
MIRGYRIKIFPNEEQKKMIHKSFGCSRFIYNWCIDRISENYNETKKTLSSIELQKEIVILKKQIEYSWLNEVSANMLKQVTIDCSNAYKRWFKLIKQNNNIKGKPRYKSRKSKQNCPTRTDRMTFNGRYVHLEKIGVVKLSKVKIDLDGKLMNARLNFDGIDYWLSFSVEYKDVQLEEKPKAEPIGIDLGLKTLVYCSNGNIYKKPHTKMIDKKIKHLQRRISKIYQPMIDYCKETRTKFSTLKKSNNLTKLEKELRKYQIRKTNILDSNIHRITSDLIKINPEKIVIEDLNVKGMMSNHKLARSIQSSKFYEIRRQLMYKCKNNNIELIVADRFYPSSKTCSSCGKIKDDLKLKDRVYRCPQCGAVIDRDLNAAINLSRIS

SEQ ID NO: 152 - protein, 379 aa, NA
MNDVIRSYKIKLYPTKEQEQLMHKHIGCCRYIWNYMINLQCSNYESGNKYMSAFTMINLLKPLKNDGEHKWLCEVSNQSLATVCQDVDKAYQRLFKKQAKKPKFKSKKRSKQAFPVRGTIWFKDNVVTIEKLGKVKFKSDFEFPQGRGNKFTNTRISEINGKWMLSFGMECENQAPELNDYSMGIDLGVKDLAIAECNGQIVFHNINKSKKMRALNKKLKHLQRAVSRKYEANKQGKKYIKTKNIEREEQKVRNIHNRISNIRNNYIHQCTHALISMLPKRVVVEDLNVKGMMKNKYLSRAIQEQCFGEFLRQMQYKCEWNGIEFVMADRFYPSSKTCSCCGVVKTNLKLSDRIYRCESCGLVIDRDYNAAINLSRYVA

SEQ ID NO: 153 - protein, 397 aa, Clostridioides difficile
MIKAIKVRLYPTKKQEVLMFKSAGISRFSYNWGLAFLNKYYEENNKFLQIDKLRKEFTRLRNNNEFSWLKEVSSEIPQQALKDLGESFKKFFKKESLYPRFKKKGKCEVSFFHLNNKFVVKENYIKLEKIGYVKMKDEGRLPIGNYKKDKIKVLNPRVKFNGKYWYLSLAMEVEEKTNIKLTNESVGVDLGIKDLAIVSNIDEPFKNINKSKEVKRLNKKLRKLQRQVSRKYDMLKSGNTFQKGEKLVKTKNIIKVEKQIKLVYKKLSDIRLNHIHQTTNTIVKTKPCRIVVEDLNVRGLLKNKHLSKSISEQCFNKFINILEYKCKWNKIEFVKADRFYPSSKMCSCCGTIKKDLKLKDRTYVCSNEKCNLVIDRDKNASINLANYKSNYKCGYLN

SEQ ID NO: 154 - protein, 331 aa, Desulfofarcimen acetoxidans DSM 771
MYAGTCVTSIFKLIKKGISKAYLLCLQMILTNGLTMSILNSKDLSGLRVYHLKHVRSLLSMRRGLLKDSLKNWVNSIPTIGWMRLKEFGYIPYGVTVKSGTVSYKAGRYYVSVIVDIQLVGVEKKCSEGIGVDLGVKVLATVSSGIKFKNINKTSKVKKLERRLKREQRKLSRKYHMRKQRGGTATALRCANIDKQRLKVQKLHQRLTNIQTDYVNKTVNELVKTKPEYITVENLNVSGMMKNRHLSKAIAQQKFYEFNIKLKSKTQWHNIELRVVDRFYPSSKICSCCGHIKWDLKLSDRIYICDNCGFVEDRDVNASINLRNAKQYKIS

SEQ ID NO: 155 - protein, 378 aa, Clostridium tetani E88
MIKALNIRLYPTQEQAALMYRHIGCMRFVYNWALARQIDSYKHSGKKLSIAELGKELTVLKNTEGYEWLYEVSNATLKEGIRDLDKAYGNFFKGRGFPKFKSKKKSEPKFYSRYEKAYFKDNLVNLEKIGKVKCKVDYDIDLTTIKKFKNPRVKFNGRVWVLSVGIEIPAKKVKLNDFSLGVDLGIKQLAITNIDNLDTLNINKTNKVKKLNKKLKKLQRQCSKKYIINKKGGSYQKTKNIGKLELKIKKLHSKLKNIRLNHTHQTTSKMVKAKPYRVVMEDLKVSNMIKNKHLSKAISEQGFNIFINQMKYKCQKYGIEFIQVSTFYPSSKTCSHCGTIKKDLKLSDRTYKCDCGFTCDRDKNASYNLANYGLEISI

SEQ ID NO: 156 - protein, 374 aa, Gracilibacillus timonensis
MMKAYKIKLNPNNKQRTLLERSAGVSRWAYNWALEQKKKRYEETGKTVSQADLRKRLTKLKQTDDYQWLFQFSNNITKQAIKDSDEAFKRFFKGQARYPRFKSKRKSKWSFYNDNHKVKRSDTHIRLEKIGWIRFAETGYLPIEFKPLSYRVSREGLHWFVSITVEIPDSSDYSTPVNEPIGIDLGIKTLATVSDGSVYVNINKKHEVRQMEKRLRRLQRQISRKYKMNKEGSRYRKTCNIIKTEKEIARLQTRLNHIRTNYIHQMTSEIVRTKPSHIVMEDLNVRGMMKNKHLADHIAKCHFREIRRQLTYKANQSGVSLVVADRWYPSSRICCECGVMDKTLKLSDRKMKCECGNRIDRDMNASINLSRLAV

SEQ ID NO: 157 - protein, 412 aa, Mitsuokella multacida
MFRGRKIRLLPTKEQELLFWKSAGTARWAYNYFLAENEAAYRAYLKRGKTGPRRISADDVRKYINNNLKKTTHQWLKEVSNNVMKMAVKKADYAVKKFLKGLAGKPKFKTKHRTKPSFYVNYASLARKNGGFHGERLGFIRTAEPLPRLPKGKRYSDPWISFDGKYWYLGLSYEVSASEAKELSGDTIGIDLGIKTLATCYVSGTKKKMTFQNINRTKKVRRLEKKLRREQRKQSRKLVANTARHKSIQREGKTIGRKPIWKRPLHECLNLKRQRRKIALIHRRLANIRQNHVHQTTATIVKTKPSRVVLENLNVKGLMKNKHLAKAIAGAKFYEFRRQMIYKCEEHGIQVIIADRFYPSSKTCSYCGYLKKNLKLNDRVYVCPSCGKAIDRDLNAAINLANYFQSDTACTA

SEQ ID NO: 158 - protein, 414 aa, Enterococcus mundtii QU 25
MSHLKIDKYNKEIEGDKDVSGVQNRNSSNRRTKKIINRTIGVARFVKNFYIYHNQEVYKSGGKFVSGIDFSKWLNNDYIPNHPDKLWIKAVYAKSTKHAIMETEKAFRNFFQGKANFPKFKKKKHQDVSMYFVKNDKKTIIRCERHRIKVPSLNWVKLNEKGYIPKHDDKHSIKSGTISQQANRYYLSVIVEQDCTAQVLNDTPTEGVGIDLGLKDFAILSTGKTYKNINKSGKIRKIEKQLKRQQRKLSRKYESEKKRVNEKQSKRGEATRKNIEKQVLKVQKLHKRLTDIRRDRVNKIVLELVKTKPAYITIEDLNVKGMMKNRHLSKAVREQSFYAFRKKLADKCKVSTIELRLADRFYPSSKLCHECGHKKVALKLSERTYRCENCGYVADRDYNASMNLKDVKEYNVIA

SEQ ID NO: 159 - protein, 391 aa, Anoxybacillus flavithermus strain DSM 2641T
MIRTYKVMLLPNNKQKTKLFQCAGVARWAYNFALAQQQENDKQGGKFLSDGELRKRLTQLKQTKEYSWLNQFSNNITKQAIKDAYQAYKNFFEGRAKFPKFKTKKRTRPSFYQDTSKIKITDTHVKLEKLTPSKKKNRQKFNWIRLAERGRIPHGAHIKYVNPRIVFDGLHWFLTVGVEEAEVKHGTYNEGIGIDLGVKSFATVSNGMTFPNIHHMPQVKKLEKQMKRMQRKISRKYEMNKIQTERGEFRYRKTENIKKLEFLVLKKRRRLKNTQLNYTHHITTTLVKTKPAYVVMEDLNTSGMLKNRKLSKAIQQQTFHEFKRQMTYKCAWHGIELIVADRFYPSSKKCSRCGHVKEKLSLSERTYRCEACGIEMDRDLNASINLKNYAK

SEQ ID NO: 160 - protein, 387 aa, Fusobacterium pseudoperiodonticum strain KCOM 1277
MYYKALKIEIKLTEEQKIQVNKTIGTERFIYNEYIKYNQEQYELGNKFVSANDFSKYINNIYLPNNPDKKWIKDVSSKSVKQAMIYGEKAFKNFFKGLSSFPVFKKKGKNELGAYFVKNNKTDFEFYRHKIKIPTLKFVRVKEYGYIPKNANIKSGTITKIADRYFLSLIIEIEDTVKATNTNSKGLGVDLGIKDTAICSNGKVFKNINKTKKVKKLKKKLKREQRKMSRSVEYSKSKKIKLKECKNFNKKKLKVQKLFYRLNCIRDDYNNKIVDEITRAKLKYIAIEDLKVSNMMKNKHLSKAIQEQNFYAIRTKLINKCKERNIELRVVNTFYPSSKTCSCCGSIKKNLKLNDRIYKCCNCGLEIDRDYNASINLEKAKIYKVIA

SEQ ID NO: 161 - protein, 407 aa, Clostridia
MEFEEQPIILFKGGLKILKSYKTEIDPTEEQTKKIKKTIGTCRFIYNFYLAKNKEIYEKSNQSMSAFSFMKWLNNEYLKENPDKLWIKEVSTVSIQKATQNATDAFRRFFKGQNRFPKFKKKNKQDVKMYFCRQGKNDSIKCERHRIKIPTLGWVKLKEKGYIPTNPNTHIIRKGTVSYKAGRYYVSVLVEEMQPMKERLNDFGIGIDLGVKEFATLSNGTIYQNINKTNRVKDLEKKLNRERRKWSRKYKSYLRRKELDENCTKENLLKQQIKMQKVFHQLDNARTDYVNKCISEIVKTKPSYITIEDLDVMRMMKNKHLSMEVQKQKFFEFRTKLADKCREYGIELRVVDRWYPSSKTCHNCGCIKHNLKLSERVYKCPECGFKIDRDLNAALNLRDSKIYKIIP

SEQ ID NO: 162 - protein, 397 aa, Lachnoclostridium phytofermentans ISDg
MKRLQRAYKVELKPTNQQIQKINQCLGVCRWLYNAYLAKNQSLYQDFKEGKLNKKKAFMSANDFDKYINNDIKVLDDCKWINDCGSKARKKAICNAEFAYKKFFKGEAQFPRFKKKGKSKVGLYFPKNNKTDFKIERHKINIPTLKWVRLKEFGYIKANANVISGTVTEQAGKYYISIVCEVEEVKNSLPKTEPLGLDLGIKDFAIFSNEIVKKNINKTSRVKKLEKKLKREQVRLSRKYECLKKQNKIRKGETTRQNIRKQIVKVQRLQQRLANIRTDYINKCVSEIVGQKPSSITIEDLNVKGMMKNRHLSKAVAGQKFYEFRIKLTNKCKQNDIELRIVDRWYPSSKLCSCCGNVKKDLKLSDRIYVCKECGLVIDRDYQASINLREAKTYMIA

SEQ ID NO: 163 - protein, 396 aa, Petrotoga mobilis SJ95
MMRLLKSYKTEINPTLEQEQQIKKTLGVCRFIYNFYIAHNKEIYEKERRFVSGMEFSVWLNNEFIPNSQEFNWIKDVSSKAVKQSIMNGERAFKKFFKGKSKFPRFKKKKNNDVKAYFPRNNKTDWTIERHRVKIPTLGFVRLKEKGYIPTNAKVGSGSVSFEAGRYYVSVLVEEDSLTAVEKGIKQDNISFSEGIGIDVGIREFVVASNGIKKKNINKSKEIKKLEKKLKREQRRLSKKYENKKKGGTATNSAKNIDKQVLKVQKLHQKLKNKRHDYVNKVVCELVKTKPEYFTIEDLNVKGMMKNRHLSKAIAKQNFHYFKIRLENKCKHLGIQLRIVSRFYPSSKICSHCGNIKKDLRLSDRVYICEECGSKIDRDLNAAINLKNAKEYAIAC

SEQ ID NO: 164 - protein, 404 aa, Lachnospira
MVWSLVKYKLEREVRKMIKTIRVMLVPNNKQKAKLFQYANTARFAYNWALGREKENHENRGKFICEGDLRKEFTQLKKKEEYLWLKKISNNVPKQAIRDACTAYQNFFNGVSKAPRFKSKKHSIPKFYQDTKKIKFTDTHVKVEGFATSKRHNKQKLNWIRLAEHCRIPTDCKHFNPRIKYDGLNWYMTVGIEYKDKESIPSNEGIGIDLGIKDLAICSDKNKYKNINKIQKVKKLEKRKRRLQRCISRRYEKNKNGECYCKTSNIKRKEKELLKVSRKLANIRLNYLHQITTEIIKRKPSFICIEDLNVKGIMKNKHLSKAIQQQCFGEFRRQIEYKSKWNNTKVIIADRFFPSSRLCSCCNKIKKDLNLSDRIYRCECGNVIDRDYQAAINLKNYGEMKISV

SEQ ID NO: 165 - protein, 313 aa, NA
MRYYLIGEFAEKIGKAIQTLRNWHKNNTFKPAYVTAAGTRYYSQEQLNNFLGLKIKTKIKDKKALIEKVGWIKINEQIPSDIKYSNPRITYDNKYWYISVGIEVNKKQENLTDISLGIDLAICSNGQVFKNINKTIKVRKLEKRLKQKQRQISRKYEMNKIKKEGGVRCQFIKTKNIEKLENTTKLIHRKLANIRNNYLHQVTTSIVKNKPYRIVIEDLNVSGMMKNKHLSDSVRKQCFYKFRQYLTYKTELYGIKLVIADRFYPSSKTCSQYSSIKKDLKLKDIVYRCPHCGAVIDRDYNAALNLSMYKSNM

SEQ ID NO: 166 - protein, 353 aa, NA
MYNYMLDLQKKRYEAGEKHLSAFSMIKLITPLKQQEGYEWLCRVSTTSMQRVCQDLANAYENFFSKRAKFPRFKSRKRSRASYPVRETVYFIDGKTQIEKIGKVVYQTNYDLPQGRGHKFSNPRISNNNGKWILTVGIECESQAPELTDKPMGIDVGVKDLAIVAFGEDQIVFHNINKSKRVRNLSRKKRKVQRTISRKYRTNGSYSKTKGIEKYERILKTIHYKLANIRSNYIHQSTHKLVSMLPKVVCVEDLNVTGMMKNRHLSRAIQEQCLGEFLRQMEYKCAWNGIELVKVDRFYPSSRTCSCCGEIKEDLKLSDRTYVCPHCGLVIDRDYNAALNLMKYAASQTRAAA

SEQ ID NO: 167 - protein, 378 aa, Clostridium argentinense strain 89G
MINLIKALNIRLYPTKEQIILMYKHIGCMRFVYNWALSKQIENYKINNKKLSVSELAKELTILKNTKGYEWMYEISNATLKESIRDLDKAYKNFFNGSSFPKFKSKKKSNHVFYTRYDRIYFKEDFVNLEKIGKVKCRVDYDIDLATITKFQNPRIHFNGRVWVLSVGIETSVEKAKLNDFSLGIDLGITQLAITNIDNLDTKNINKTNSVKKLNKRLKRLQRQCSRKYEKNKEGGSYQKTKNIVRLEKKIKKLHSKLKNIRLNHIHQSTSKMVKAKPFRVVMEDLKVSNMMKNKHLSKAIAEQGFNKFINQMKYKCEKYGIEFIQVPILYPSSKTCSHCGYIKKDLKLSDRIYKCSCGFSCDRDKNASYNLANYGLV

SEQ ID NO: 168 - protein, 376 aa, Acetoanaerobium sticklandii strain DSM 519
MIKSIKIRLKPTKEQEILMFKSVGVARFAYNWGLAKWEEMYKKGLKPSKAKIRKEFNNSVKKSDDFKWLYEVSGQITSQAFTDLEYAYKNFFNKTSDKPKFKTKKKSKKSFYVRYDALKFKDAKVNIEKIGKVKYSSNYNIPQLDNYVNPRCHFDGKYWYLTFGFEHSENKAKLDYNLSIGIDLGIKELAYVSCFNKPIKNINKSVKVKKLKKRLIRLQKQVSRKYEANKSGDRYNKTSNIIKLEKQIKLLHRKLNNIRNNHLHQTTKMIVKLNPYRIVMEDLNVTGMMKNKHLSKAIAEQKFYEFIRQIKYKCEFNNIEFLQVDRFYPSSKTCSSCSGIKQDLKLKDRIYHCDKCGLTMDRDKNASINLANYKIV

SEQ ID NO: 169 - protein, 409 aa, Mitsuokella jalaludinii
MLRGKKIRLLPTPEQEILFWKSAGTSRWAYNYFLARNEEQYKTYLANGRKGKKSISEGVIRKEINNQLKPITHQWLKEVGSNVMKQAVKEAGRAMKKFLSGAAGRPKFKTKRRTTPRFYVNYESLTRKNGGFHGEKIGFVRTAEPLPKIPKGCHYSNPWISFDGKYWYIGFGYEVPDRLNVELTGDSIGIDLGVKELAVCYAFGERKKTVFKNINKTKEVHRLEKKLRREQRRQSRKFTANIDHYETVQRNEKKTGRRPIWKRPIRECRNIERQRQRIILLHRRLKNIRENHIHQTTAAIVKTKPSRIVMEDLNVKGMMKNRYLAKEIASEKFYEFRRQMEYKCEPYGIQLVFADRFYPSSKTCSHCGHIKKDLKMNNRTYICPACGHVIDRDLNAAINLAKYFKSEIA

SEQ ID NO: 170 - protein, 409 aa, Mitsuokella multacida
MIVGKKIRLHPTSEQETLFWKSAGTARWAYNYFLIRQEEVYQEYLVNGQKGRRGISEGTVRKEINRVLKPTTHAWLKDIGSNVMKQAVKTADKAWKKYLKGLAWKPKFKSKKMTKPNFYVNYESLSRKNGGFHGEKIGFVRTAEPLPKLPHKKHYLNPWISFDGKYWYLGFSYEVEAHRESLTGDHIGIDLGVKSLAVLYSVDTGQSKVIKNINKSRKVLRLEKKLKRAERKRTRQLKSNVLRYEPIQRDGKRPGRKPVWKRPVPECKNIEKQRRKIKLIYRKLKNIRVNHLHQATTAIVKTKPSRVVLETLNIQWMMKNKHLAKAISKAKLYEFRRQIEYKCQKCGIEVVFADKFFPSSKQCSSCGEIHHELTLSDRMFSCSCGLHIDRDLNAAINLARYTPSKIAHN

SEQ ID NO: 171 - protein, 409 aa, Mitsuokella sp. AF21-1AC AF21-1AC.Scaf4
MLRGKKIRLLPTPKQEVLFWKSAGTARWAYNYFLGENQAVYKAYLEHGKVGPKRISEGAIRKHINNELKKTTHQWLKEVGSNVMKMAVKEADRALKRFLKGIAGKPRFKTKHKTKPSFYVNYESLVRKNGGFHGEKIGFVRTRETLPKLPKGNHYCNPWISFDGKYWYLSFSYEVPEQETEKLTGDSMGIDLGIKVLATCYASGERKATVFKSVNKTKEVRRLEKKLRREQRKQSRKILANTARYETVQRKGKKPGRKPIWKRPLRECQNIEKGRRKIALIHRRLANIRQNHIHQTTAAIVKTKPSRIVMEDLNVKGMMKNKHLAKGIAGEKFYEFRRQMTYKCENNGIQLVFADRFYPSSKTCSCCGHVKENLKLNDRKYVCQACGTTIDRDLNAAINLANYFQSETA

SEQ ID NO: 172 - protein, 301 aa, Eisenbergiella sp.
MPAQPIKTFSRVYNGTQGLRRKRNQCLNSIKIQFRDTHVKFEGFSFSRKANKQKLNWVKLAEHGRIPTDAKYRNPRVSFDGLNWWISVCVEFPDCRDRSNHDGIGIDLGIKNLAICSDGNTYKNINKSQTVKKLEKCKRRLQRSVSRKYEHNKKGGSYCKTNNIVKKEKLLLKVNHRLANIRKDYLNQTTSEIVNRKPRFICIEDLNVSGMIKNRHLSKAVQNQGFFEFRKQLEYKCNDRGIQLIVADRFYPSSKRCSCCGKIKKDLRLSDRTYKCECGNVIDRDFQASLNLKAYGEQFAS

SEQ ID NO: 173 - protein, 387 aa, Finegoldia magna ATCC 29328 plasmid pFMC
MLITYKTEIKPNPEQVIKIKQTMGVCRFIYNFYIVENQKAYKNNMPFITAFNFSKWLNNVFIPNNLNYSWIRDVSSKSVKQSIVCAERAFKRFFKKESKFPRFKKKNKSNVKMYFVRNNKGDCLCERHRIKIPTLGWIKIKEKGYIPTSKDDYVVKSGAISYKAGRYYISCLVDIEEPPKQILKPFGLGIDLGLEKFAVISNGNVYKNINKSKKIIKLEKKLRHEQKCLSRKYEQLKNNKKGESTHKNILKQIAKVQKTHLKLSNIRTDYINKIINELVKTKPAYIVIENLNISGMIKNRYLSKSISNQRFYEFRQKLFNKCNFHGIELRIADRFYPSSKTCHSCGSIKKDLKLSDRIYKCPTCGEIIDRDLNASLNLRDTTSYKIA

SEQ ID NO: 174 - protein, 392 aa, Clostridium aceticum strain DSM 1496
MKKMIKGIKVMLIPNNKQNTKLFQYAGASRFAYNWGLAKQQENYKNSGKFINDGELRKEFTQLKKQEGYEWLNNISNNVTKQAIKDACNAYKRFFKGESKFPRFKSRKKSAPKFYQDVEKIQFNGTHVKFEGFSTSKKKNKQKLNWVRLAEYNRIPFGENEKYINPRVSFDGLNWWVSVGIEHEDEVKQPTNEGIGIDLGIKDLAICSDIDKPYKNINKTSKVKKIKKKLRRLQRKISKKYEMNKEGSRYKKTCNIIKLENKLKKVHHQLKSIRHNYIHQTTCEIVNREPMFIVLEDLAVSNMMKNKHLAKAIGEQCFYEFYRQIEYKALWNNVKFIIADRFYPSSKMCSVCGAIDKDLKLSDRTYICECGNKIDRDKNASVNLKNFGELAI

SEQ ID NO: 175 - protein, 391 aa, Eubacterium sp.
MLKSYKTEIDPTPEQKQHISRTIGVCRYVYNFYLAHNQEIYEVEKRFVSGMDFSKWLNNEFIPNNPDFHWIKEVSSKSVKQSIMDAERAFKNFFKGKSRFPRFKKKARSDVKMYFVKTDAKVIIKCERHRIKIPTLGWVRLKEKGYIPTNPKTHIIKSGAVSCKAERYYVSVLVEEQEPQKPVLNDFGIGIDLGLKDFAVCSNGKTYKNINKSSQIRKLEKKLKREQRSLSRKYESYKKLNKNMKGVATRQNIQKQKLKVQELHQRLDNIRTDHIKKVVSELAKTKPMWITIEDLNISGMMKNRHLSKAIAQQKLFEFRTKLLAKCNSYGIELRIVDRFYPSSKTCHNCGSVKSDLKLSDRTYHCCECGYAEDRDYNASLNLRDCRTYKIA

SEQ ID NO: 176 - protein, 392 aa, Monoglobales
MLITKKIRLKPTTEQEILFRKSAGVSRWAYNFFLGENKRIYREYIDNGKVGKKSISEGDVRKYINNVLKPTTHSWLKEVGSNVMKQGVKDANLALQRYFKDLSGKPKFKSKHKDRPSFYVNYESLSRKQGGFQGEKIGFVKTSESLPKLNKNEKYSNPRITFDGKYWYLSVGYEAKENTVELTDESLGIDLGVKDLAICSNGKVYKNINKTQRVKNLEKKLKREQRKLSRKIENNIQSYKSNRSPVYKRPLKECQNVQKQNRLIRNIHRKLANIRQNYLHQTTTEIVKTKPSRIVMESLNVSEMMKNKHLSKAIQQQKFYEFKRQIEYKSKLNGIEFIQVDKFYPSSKTCSCCGNIKKDLKLSDRMYKCDVCGLVIDRDYNASINLANYEVI

SEQ ID NO: 177 - protein, 371 aa, Intestinibacter bartlettii
MILAKKVRLCPSELQEEKLWQSVGTARFIYNWALNRQEENYKGGGKFIPDSVLRKEITQLKKTDLSWLNEVSNNVAKQAVKDACDSYKRFFKGLSGKPRFKSRKRSKKSFYHDNVKLKVKDNKLVKIEKIGWIKTNEQLSIGAKYSNPRISYDNKYWYLSVGIEQEEIQEELTDASLGIDLGLKNLAICSDGTVYKNINKTCTVKKIEKKLKRLQRQVSRKYEKNKKGKEYVKTKNIIKLEKQIQQTHRRLANIRNNYLHQTTTSIVKTKPYRVVIEDLAVSNMMKNKHLSDAIRKQGFYEFRRQLEYKCNFRGIKLVVADRFYPSSKICSQCGEIKKDLKLSDRVYKCNCGLVIDRDLNASINLSKYKLA

SEQ ID NO: 178 - protein, 399 aa, NA
MNEEDKGDQERMLKSYKTEINPTMEQIHKINKTIGTCRFVYNFYLARNKEVYEKEKKFVSGMEFSKWLNNVYLKENPEYVWIKEVSTKSVKQSIMNSERSFKRFFKGQSGFPKFKKKGKSDVKMYFVKTNSQTIITCERHRIKISTLGWVRLKEKGYIPWDSNTYIIKSGTVSCRAGRYYVSVLVEQPERERLQLQDFGFGIDLGVKNFAVISNGLVKKNINKTNKVKKLEKQLKREQRCLSRKYESLKKNNKKGESSRENIQKQILKVKRLYCRIDNIRTDYINKTIAEIVKTKPSYIAVEDLNVSGMMKNRHLSKAVASQKFYEFRVKLEAKCKEYGIELRIVDRWYPSSKLCHECGCIRKDLKLSDREYVCECGYHADRDYNASLNLRDATSYKVA

SEQ ID NO: 179 - protein, 371 aa, Clostridium sporogenes strain CDC_1632
MILAKKIRIIPNMEQEQQLWKSVGTARFIYNWTLARQEGNYKNGGKFIKDGDLRKEITIMKQTEEYKWLKEVSNNVAKQAVKDGCNAYKRFFKGFADKPRFKSRKKSRPSFYNDNLKLKVKPKMALIEKVGWIKTAEQVPMNIKYTNPRVSFDGKYWYLSVGVEKENSKVELTGESIGIDVGIKDLAICSNGMTFKNINKTRLVKKLEKRLRRLQRKISKKYELNKEGRKFVKTSNIIKLEKQIRLLHRRLSNIRNNYLHQATTKIVKNKPSRVVMETLNIKGMMKNRHLSKAIAQQGLYEFKRQLQYKCEFYRIEFVEADKWYPSSKICSECGHKKTKLSLSERTYICEECGVVIDRDFNASINLSRYSA

SEQ ID NO: 180 - protein, 379 aa, Clostridium novyi strain 150557
MKMILLKKVRLYPTGIQEQKLWQSVGTARFIYNWTLNKQQENYKNGGKFIKDSDLRKEITLMKKTDEYKWLSEVSNNVAKQAVKDCCNAYKNFFKGLSDKPRFKSRKKSKPSFYNDNVKLKVKTKLVNIEKVGWIKTKEQIPINVKYTNPRISFDGKYWYITVGVEQEQSTIELTNKSIGIDVGIKDLAICSNGMTFKNINKSKEVKRLKKVLKRKQRKVSRKYDMNKKIEGGENRCQYKKTNNIIKLEKEIRLLHRRLRNIRNNHIHQATNKIVKTKPSRVVMETLNIKGMLKNKHLSKAISEQCLYDFKTKMQYKCKLYGIEFIEADKWYPSSKTCSCCGAIKKDLKLSDRVYKCKCGLVIDRDLNASINLSRYKLA

SEQ ID NO: 181 - protein, 373 aa, Clostridium sporogenes strain AM1195 plasmid pRSJ11_1
MILGKKVRLYPTKDHEQKLWQSVGTARFIYNWTLARQEESYKNGGKFISDNDLRKELTILKKTELNWLNEVSNNVAKQAVKDGCEAYKKFFKGLADRPRFKSRRKSKPSFYNDTSKLKVKENSVLIEKVGWINIKKNSIPMNCKYSNPRISFDGKYWFIAVGIEKEKPIVELTTESIGIDVGVKDLAICSNGMTFKNINKARVVKQLEKRLRRLQRRVSRKYLKNKEGSKFVKTSNIIKIEKQIKLLHRKLANIRSNYNHQATNKIVKTKPSRVVMETLNIKGMMKNKYLSKAIAKQCLYEFKKQMQYKCEFNGIKFVEADKWYPSSKTCSECGHIKPKLSLSERTYICEECGCVIDRDYNASINLSRYELVG

SEQ ID NO: 182 - protein, 388 aa, NA
MIILLKSFKTEINPTAEQIIKINKTIGVCRFIYNFYIAHNKELYENGEKFISGRRFNVWLNNEYLPNNPDKMWIKDVYTKAVAKSMDNACVAFTRFFMCKSKFPRFKKKNKSDVKMYFVKNNKTDCLSERYRIKVPTLGWVRLKEKGYIPTSKDGFIIRSGTISHKAGRYYISVLVDIEKQDTEMSNNFGIGIDLGLKSLAVCSDGSTYCNINKTYNIRKVEKILKREQRKLSRKVISIKKGESTRKNFVKQRLKVQKLYQRLDNIKTDYINKTISKVVKTKPSYIVIEDLNVSGMMKNRHLSKAVAQQKFFEFKTKLISKCKENNIELRVVDRFYPSSKLCHNCDNVKKDLKLSDRIYKCSECGYVEDRDINASLNLRDAKTYTIIQ

SEQ ID NO: 183 - protein, 372 aa, Bacillus thuringiensis BMB171
MMLAKKVRIKPNKGQELQLWKSVGTARWAYNWTLAKQEENYKNGGKFISDVFLRKELTVLKQTEEYAWLYDVSNNIAKQAIKDACEAYKRFFKGLADKPRFKSRRKAKLSFYNDNVKLKVKEKQVLIEKVGWVKTSEKLPVGVKYSNPRVSFDGKYWYLSVGIEQEFTKEKLTAVSLGIDIGIKELAYCSDGQRKNNINKTKMVRQVEKRLRRLQRQVSCKYEMNKEGNRFVKTSNIIKIEKEIRQLHRRLSNIRKNHLHQSTSEIVKTKPFRIVMETLHMKGLMKNRYLAKAIAKQCLYEFKRQIQYKCEKYGIEFVEADTWYPSSKMCSSCGSINKELKLSDRVYKCTCGHEMDRDLNAAINLSRYELAS

SEQ ID NO: 184 - protein, 372 aa, Bacillus thuringiensis serovar chinensis CT-43 plasmid pCT14
MILVKKVRLKPNREQEMQLWKSTGIARWAYNWALSRQEENYKQGGKFISDGTLRKELTQLKQTEEYAWLYDVSNNVTKQAVKDLCEAYKRFFKGVVDKPRFKSRRHSKPSFYNDNVKLKVMKNMVLIGKVGWVKTSECIPVVNKYSNPRISFDGKYWYLAVGIEQEIIHQELTNASIGIDVGIKELAFCSNGMKFKNINKTKVVKQVEKRLRRLQRQVSRKYEINKEGSCFVKTSNIIKLEKKIQHLHRRLTNIRDNHIHQVTCAIVKTKPCRVVMETLNIKGMMKNKHLSKAIAQQKLYDFKMKMKYKCEKYGIEFVEADKWFPSSKQCSNCGEVNKHLTLSDRTYHCKCGHHIDRDLNASINLSRYQLVN

SEQ ID NO: 185 - protein, 397 aa, Anaerostipes hadrus strain BPB5
MMVVKKMIKTIRVMLIPNNKQNTKLFRYANTARFAYNWALGREKENYKNGGKFLSDSDLRKEFTQLKKTEEYSWLKEVSNNVTKQAIKDACHAYKRFFKGCSKFPKFKSRKFSIPSFYQDNVKIQFSDTHVKIEGFAASKKKNKQKINWIRLAEKNRIPTDCNYSNPPIRYDGINWWITVGIEYEDSVTVPSNDGIGIDLGIKDLAICSDGNKYKNINKTKKVKKLEKQKRRLQRSISRSYENNKQGKEYCKTKNVIKKEKLLLILNHRLTNIRHDHLHHITSEIVKREPSFICIEDLNVKGMMKNRHLSKAVQQQGFYEFRRQMEYKSKWNNIQAIIADQFFPSSKLCSCCGKIKKDLKLSERIYKCECGNVIDRDLQAALNLKKYGEDVLKRSVA

SEQ ID NO: 186 - protein, 385 aa, Erysipelotrichaceae
MYKSFKTEINPTPTQKAKIDKTIGTCRFVYNFYLAHNIELFNAGEDLMTGKMFSVWLNNEYLPNNPEYNWIKDTYSKAIKKSIEDGFTSFKRFFKHESDFPRFKKKGKSNVKMYFVKNNKTDCKCERHRIKIPTLGWIRIKEKGYIPTEKQGWNIKSGTVSYKAGRYYVSVLAEIPDIEYEKTSNEGVGIDLGIKDFSVISNGNVHENINKSHKIRKLEKKLRREQRCFSRKYENLKKEGEPTQKKNIEKQKLKVQKIYHKMDNIRTDYINKTIAEIVKTKPSYITIEDLNVKGMMKNKHLSKAIASQKFCEFRRKLKIKCDNQNIELRIVDKFYPSSKLCHHCDSIKKDLKLSDRVYRCKCGYIEDRDRNAALNLKDAQSYVVA

SEQ ID NO: 187 - protein, 370 aa, Paenibacillus durus ATCC 35681
MILTKKVRIRPALEQEQQLWRSVGTARWVYNWTLSRQEENHKHGGKFLSDGDLRKELTQLKHTEEYAWLCNVSNNVAKQAVKDACDAYKKMFKGLAKKPKFKSRKKSRPSFYNDTAKLKVKDQVVLLEKVGWMKTVEQLPIGVSYSNPRVTFDGKYWYLSVGINQEQVQQKLTDEVVGIDVGVKELAVCSNGMVFKNINKSAAVRKTEKRLRRLQRKVSRKYEMNKEGSRFVKTSNIVKVEKSIRLLHRRLTNIRTNHIHQATSAVAKTKPRAVVMETLNVSGMMKNRHLSQAIANQKLNEFIRQMKYKCEKRGATFMQADRWFPSSKCCSGCGQVKTHLKLSDRIYECDCGLKIDRDLNAAINLAQLAV

SEQ ID NO: 188 - protein, 390 aa, Clostridium sp. JN-9
MKKLKKAYKTEIKPTKEQIIKIRRTIGVSRFIYNFYIAHNKEVYEKEKKFVSGMDFSRWLNNEYIPNNQDKVWIKKVSSKAVKQAIMNGEKAFKKFFKGEAGFPKFKKKKNQDIKAYFPKNNETDWTIERHRIKIPTLGWIGLKEYSYIPANGRITSGTVSQKADRYYVSVLVDEDIKINNKRCSEGIGVDLGLKDFAICSNGITKKNINKTKTVKKAEKKLKREQRKLSRKYESLKLRNKKEKGEATRQNIQKQIVKVQKLHQRLTNIRTDYINKTVSELIKQKPRFITIEDLNVRGMMKNRHLAKAVAQQKFYEFRIKLISKSKQDGIEVRIVDRFYPSSKTCSCCGRIKKDLKLSDRVYKCDNCNTSIDRDLNASINLANAKEYKIA

SEQ ID NO: 189 - protein, 433 aa, Selenomonas ruminantium subsp. lactilytica TAM6421 plasmid pSRC1
MIRSVRIRLLPNNKQRTKLFQFAGASRFAYNWALDKQMENFREGRKLQSDYDLRKEFTVLRNSEEYLWLLGISNNVTKQAIKDLCIAYKNFFHKQRQKGYVKYSPKKLAHFARIARTPTIYDMNGHPKFRSKKNGDFRFYQDNVKIQFTATHVKLENIAGSRKKNRQRLNWIRLAEKGRIPTKGRYTQPRITFDGENWWLSVGIRTSYTLKPMRGLNFSRKQPGRFCTEGVGIDLGIKDLAIISDSTVVKNINKSHTIRNIKKKRRRLQRQVSRKYQMNKKGERYCKTSNLIKSEKRLLRINHRLADIRANHVHQATRIIINRKPRFICLEDLNVQGMMKNKHLSEKVQEQNFYEFRRQIEYKAHWARIPVVIADRWFPSSKTCVECGYINKDLKLSDRTYVCPVCGNVIDRDFQASLNLKRYGETELSKSAS

SEQ ID NO: 190 - protein, 393 aa, Blautia wexlerae
MMIKTIRVMLVPNNKQKTKLFQYANTARFAYNWALGREQENYKNGGKFISDGDLRKEFTQLKKKEEYAWLNYVSNNVTKQAIKDACEAYRDFFKGYTKFPRFKSKKHSVPKFYQDNVKIQFTDTHVKVEGFATSRKKNKQKLNWIRLAEHGRIPTEKVKYMNPRIKYDGLNWYITVGIEYEDSTTLSTNEGIGIDLGIKDLTICSDGNTYKNINKTHKIKKLEKRKRRLQRSISRRYEKNKKGGSYCKTSNIIKSEKELLKLNHRLTNIRQNYLHQTTTEIVKTRPSFIVLEDLNVKGMMKNKHLSKSVQQQCFGEFRRQIEYKSAWNNIQVIIADRFFPSSKLCSYCGNIKKDLKLSDRIYRCECGNVIDRDYQAALNLKKYGEMALEQSVA

SEQ ID NO: 191 - protein, 370 aa, Brevibacillus brevis strain DZQ7
MILAKKVRLKPTPEQERQLWKSVGTARWAYNWTLAKQEENYRNGGKFLLDGDLRKELTQLKQSEEYSWLYEVSNNITKQAVKDACDAYKKFFKKLAEKPTFKSRRRSKPSFYNDNVKLKVKQNHVLIEKVGWVTTSEQLPTDVNYTMPRISFDGKYWYLSVGVEQEFIQPELSGESLGIDVGVKELAVCSNGMTFKNINKTKVMKKAEKRLRRLQRKVSRKYEMNKEGSRFVKTCNIVKVEKHIRLLHRRLTNIRTNHSHQATSAIVKTKPSTVVMETLNIKGMMRNRHLSKAIAQQKLYEFKRQLQYKCEKYGIRFMEADKWYPSSKTCSDCGEVKKDLKISDRIFKCVCGLVLDRDVNASINLAKLAS

SEQ ID NO: 192 - RNA, 256 nt, synthetic construct
  source 1..256: mol_type = other RNA
taaaaccatagttataaggacttcacatgacctaaaacattatagtacaatgaataatgagaccaattaacccgttatgtctccaaaaactaccgttggttctaccgtgggttggcaggtaagttacgcacgtggactgttacatcaaaccgtagtagacactccttgcagtttcgagacgggacaggaagaagcgtgaaaaagctcaaccagataatgataatatgcgtatggttgagttactggcatggaacag

SEQ ID NO: 193 - RNA, 139 nt, synthetic construct
  source 1..139: mol_type = other RNA
tttatataaaatagtgagactgctctcacgaatttaagcctatggagagttaaaaccacttgagtagttgcgacgaaaaagaattcgaagaagtaggaaatattagaatatacaactttgtataagtttaatatagcag

SEQ ID NO: 194 - RNA, 207 nt, synthetic construct
  source 1..207: mol_type = other RNA
atagagaggctataacctcaaggtgtcgttgcacctttaagctgtggagtgttatataaacttgagtaggattacccaaaagaggacgctgagaagcagtaagttagattggctaacacaacggaaaaggaatgatttatatggttaaaatctcgcaggaggaagcttttaagattagaaagaagtttccgggaacgcatataacgg

SEQ ID NO: 195 - RNA, 184 nt, synthetic construct
  source 1..184: mol_type = other RNA
catagaaaatcaaataaaaagattgtgctaatatgtagacattgacgaggtcgaatttaagcctttggactgctacattaaactagagtagaaattgaatttcaaaatagagcaggaggaaaaaggaaataaaactataaaaaatataaagtatttatataaatttatagagtttatacgtcag

SEQ ID NO: 196 - RNA, 153 nt, synthetic construct
  source 1..153: mol_type = other RNA
ttaacaaagttcttgtatatgtaccgatggctagtcgggaatttaagactgtggagtgttacatcaaatgcgagtagctttgtggcaaaagcagacattatgaagcagtaaaactctcttgatatagatttttgtctatatttaaagtagcag

SEQ ID NO: 197 - RNA, 167 nt, synthetic construct
  source 1..167: mol_type = other RNA
aaagatattctaaattgggtaatcgttacaacccattaccttgctaggtaacaaagcctatggagtgttatagcaaacgaaagtagcttaggcaaaatcggatattatgaagtaggaaagaaacaaaaatctttaatttatagatttttataggtttttggtaacgg

SEQ ID NO: 198 - RNA, 170 nt, synthetic construct
  source 1..170: mol_type = other RNA
tcacgaacaagacacggctaataggtaccgtgagttacacgggaatgaacgccctcggagtgttacagcaaacgagagtagtatctgagacagatacaaaatcggacacggtgaacagggaagaaaacaaaaaatctcttttacaggtttttataagtttttcgtaacgg

SEQ ID NO: 199 - RNA, 212 nt, synthetic construct
  source 1..212: mol_type = other RNA
aacttagagaaattctcagacaggtacctatcgctactagggaaccggctttcctaaaaagattgtctaagcctgcggagcgttatatcaaacgtgagtagccatcgagcttgcttgaggccaaaacggacgcgatgaaccaggaagaaaacatcgcaagagttttcgaagtataactctgtatgataatttatacagatttatcgtagcga

SEQ ID NO: 200 - RNA, 177 nt, synthetic construct
  source 1..177: mol_type = other RNA
gcacgcaactttgtatatgtaccgatggcttagtcgggaatcaacgactgtggagaacgagacaaaccgtagtagtgtcgaagtgacgaggcggcgttcggtgaaacagtaattctacctacgtgagtggtagagaaatctcgatataggtatttttgtctatattttgtgtagcag

SEQ ID NO: 201 - RNA, 154 nt, synthetic construct
  source 1..154: mol_type = other RNA
agcacaacatgtacccatccgttagtggggaagtgaagccttcggagcgccaaggaaacgagagtagcttcggcaaaatcgggcgcgatgaacaaggaaggaaacatagacttttataggtttcttataaagtcttgtaagttttctgtaacgg

SEQ ID NO: 202 - RNA, 157 nt, synthetic construct
  source 1..157: mol_type = other RNA
caagttaaaatatctatatgtaccgatggctagtcgggaatttacgactatggagagtacaaggaactatgagtagatactaagtattgaaaatatactcgttgaagtagtaacattctagtgtattaaatatgttttaatacatttatagtagcag

SEQ ID NO: 203 - RNA, 168 nt, synthetic construct
  source 1..168: mol_type = other RNA
ctaatctgtaaatatgtaccgatggtttgtcgggaatttacgactgtggagtatactagaacttgtgagtagcgtgttattcgtaaccgcaaaagcatatacgaagaagcagtaagaggtatctgtaaaaccctcaattctcaatacttatgtattttagagaaacag

SEQ ID NO: 204 - RNA, 160 nt, synthetic construct
  source 1..160: mol_type = other RNA
ccacgttactgtaagtatgtacccaaggctatttggggaatttacgccctcggagtgttatagcaaatgagagtagtgtattataacaatcaccaaatcagacacgttgaacagggaataatctcgatatgggtagatttgtccatattttgagtggcag

SEQ ID NO: 205 - RNA, 149 nt, synthetic construct
  source 1..149: mol_type = other RNA
aattgctttgcatatgtgtaccgatggccagtcgggaattcacgcctgtggagtgtcaaacaaaccgtagtagatatatatcgaggcgggacacgttgaagcaggaaacttctggatataggcatgtttgtctatgttttcagtggcag

SEQ ID NO: 206 - RNA, 172 nt, synthetic construct
  source 1..172: mol_type = other RNA
aacacgaaaaagttaatacagatgtgtacgaatacgttagttcggaatttacgcctatggagtgtacaaggaactgtaagtagtaactaaatttatttagtacaaaagcatacacgatgaaataggaatgaaacataaaagtttataacttgttataagttttcagtaacgg

SEQ ID NO: 207 - RNA, 125 nt, synthetic construct
  source 1..125: mol_type = other RNA
gacacgttgtatccaaatttaagcctttggagaatcatatcaaacgaaagtagctatggcaaaatcggattctatgaagaaggaagtaaacaaatttatatattgttatagattgttggcaacgg

SEQ ID NO: 208 - RNA, 212 nt, synthetic construct
  source 1..212: mol_type = other RNA
gggaatcgttgcacccctgaatgctgtggagtgtcatacaaacccgagtagctaaggccaaaggggacacaatgaagcagtgattggaattaccaaacgcaacggtacaacgtgctggatgtagaggtcatggctaagattctctatcgggaagctcgtggcatctccagcaagacagaacaggcctgcgtcggctgggtgatctgtaacag

SEQ ID NO: 209 - RNA, 188 nt, synthetic construct
  source 1..188: mol_type = other RNA
tcaattaaaagattaactaaattggggaatcgttataacccactaccttattattaggtagcaaagtctatggagtgttatatcaaacgaaagtagcttaggcgaaatcggacattatgaagtaggaaataaacaaagctataaacttatataatctttttatagagtttttagtattttggtaacgg

SEQ ID NO: 210 - RNA, 178 nt, synthetic construct
  source 1..178: mol_type = other RNA
ttttgaaaaattatactatatgtatcctgcgttgtgggagaatttaagtccttggagagttacaccaaactaaagtagagtgagaaatcattcaaaatagaactcgatgaataggaaatgttatttggtaacaaataatgtaagtaaaatttatatatttataagttttatgcaacgg

SEQ ID NO: 211 - RNA, 197 nt, synthetic construct
  source 1..197: mol_type = other RNA
catttcgagaagcacttagatatgtacctatcgctactggggaatttaagcctgtggagcgttatatcaaacgaaagtagctgcctgcttcggcagggcaaaatcgaacgcaatgaaacaggaaggatgtttgtgaaaacattcaaagtgtaaatttgtatagtataaaatagatatttacagatttatcgtagcgg

SEQ ID NO: 212 - RNA, 179 nt, synthetic construct
  source 1..179: mol_type = other RNA
gagcagtttcgatatgtacctatcgctgctggggaatttaagcctgcagagcattatatcaaacgagagtagcttgcaatgcgttgtggcaaaatcggatgcgatgaagcaggaagagtgctcgtgagagcagtcaacgtattgatttatgatatatatcggtaaatcaatcgcagcgg

SEQ ID NO: 213 - RNA, 200 nt, synthetic construct
  source 1..200: mol_type = other RNA
aatacagagaagcactcagatatgtacctatcgctactggggaattcaagcctgtggagcgttacatcaaacgcgagtagccatcgagcttgctcgggggcaaaaacggacgcaatgaaacaggaagaaaatatcgtgagaattttcatcgtataaatttgtgcgaattatattatatttatacagatttatcgtagcgg

SEQ ID NO: 214 - RNA, 168 nt, synthetic construct; identical to SEQ ID NO: 88
  source 1..168: mol_type = other RNA

SEQ ID NO: 215 - RNA, 159 nt, synthetic construct
  source 1..159: mol_type = other RNA
taaaaaaagctatataagatatgtaccgatggctagtcgggaattgacgactgtggagtgtacaagaacttgttagtagcaaaatctttgcaaaagcatacacaatgaagcagtaatttatctcgatgtagacttatttgtctatgttttgagtagcag

SEQ ID NO: 216 - RNA, 163 nt, synthetic construct
  source 1..163: mol_type = other RNA
tcacttaaaagatattgctaatatgtactcatacgttaatgaggaatttatgcctttggagtgttatatcaaacgaaagtagcataggcaaaatcggacacgatgaacaaggaaagaaacacaaaagtttattttataactttttataagttttctgtaacgg

SEQ ID NO: 217 - RNA, 151 nt, synthetic construct
  source 1..151: mol_type = other RNA
acaagctaatgtaggtatgtaccgtaggctatacgggaatttacgcctgtggactatacaagaacttgtgagtagtcttaggacaaaagcatataggttgaagcaggaattttctcaatatgggtgtatttgtccatattttgagtagcag

SEQ ID NO: 218 - RNA, 190 nt, synthetic construct
  source 1..190: mol_type = other RNA
attcacttaaaagaattatataactatgtacctatcgctattagggaatttacgtctatggagtgtcataacaaatgaaagtagctacggcaaaatcagacacgttgaagtagaaagtcttaatcgtgagataagacacagtatagatttatatagattagttgtaatttatatatatttatcatagcgg

SEQ ID NO: 219 - RNA, 168 nt, synthetic construct
  source 1..168: mol_type = other RNA
tatcattaataagataatgctaatatgtaggatgcgttgtatccgaatttacgcccttggagagttatatcaaacgaaagtaggttgttatttataatttccaaaatcgaattcgtagaacagggaattaaacaagatttatagatatttatagatttttggcaacgg

SEQ ID NO: 220 - RNA, 184 nt, synthetic construct
  source 1..184: mol_type = other RNA
acaagcatttgcaggtatgtaccgatggctagtcgggaattgacgactgtggagtgtacaagaacttgtgagtagtatctgtatttactcagggcgaaagcatatacagagaagcagtaagaaatgttcgcaagaactttcaatatctcgatatggatatctttgttcatattttgagtagcag

SEQ ID NO: 221 - RNA, 154 nt, synthetic construct
  source 1..154: mol_type = other RNA
ctacttaaacagttatgtttgaggtgtaggattcgttgtatccgaagttaagccctcggagtgctatacaaaccaaagtagctacggcaaaatggagtacgttgaacagggaattaaacaagctttatagagttttataaggttttggcaacgg

SEQ ID NO: 222 - RNA, 156 nt, synthetic construct
  source 1..156: mol_type = other RNA
tatcacttaaaaagataatgctaatatgtaccattcgttgtatgggaatttaagcccttggactgttatacaaaccaaagtagcctcggcaaaatggaacaggtggaacagggaattaaacaaggtttatagatatttatagatttttggcaacgg

SEQ ID NO: 223 - RNA, 156 nt, synthetic construct
  source 1..156: mol_type = other RNA
tcacttaaaagatactactaatatgtaccatgtgttgtatgggaatttaagccctcggagtgttatagcaaacgaaagtagctttatagcaaaatcggacacgttgaacagggaattaaacaagctttatagagttctataatgttttggcaacgg

SEQ ID NO: 224 - RNA, 184 nt, synthetic construct
  source 1..184: mol_type = other RNA
atatagtgtataagtatgtaccaatggctagttgggaatttacgactgtggagtatagaagaacttgtgagtaatatattcaactttgttgaattatgaaagcatatacgttgaagcagtaagtaaaaatcgtgaggttttacaattctcattatagacattaggtctataatttgagtagcag

SEQ ID NO: 225 - RNA, 155 nt, synthetic construct
  source 1..155: mol_type = other RNA
catctaaaaaagttacggctaatatgtaggattcgttgtatccgaatttacgccctcggagtgttacatcaaacgaaagtagcttctgtgaaatcggacacgtagaacagggaaataaacaaaatttatagatttttataagtttatggcaacgg

SEQ ID NO: 226 - RNA, 153 nt, synthetic construct
  source 1..153: mol_type = other RNA
cactaaaacgttattgctaatatgtaggattcgttgtatccgaatttacgcccttggagtgttatgtcaaacgaaagtagcttcggcaaaatcggacacgtagagtagggaagtaaacagactttataaagttttataaggttttggcaacgg

SEQ ID NO: 227 - RNA, 170 nt, synthetic construct
  source 1..170: mol_type = other RNA
tatattcaagtgattacagatatgtactgatacgttagtcaggaattaacgcctatggagagtacaggaacttgtgagtagtacatgaattgattcgttacaaaagcatactcgttgaagtaggaatgaaacataaaggtttataactttttataagttttcggtaacgg

SEQ ID NO: 228 - RNA, 187 nt, synthetic construct
  source 1..187: mol_type = other RNA
aagatagaaaagaattttaagcatgtaccaaaggctaatttgggaattaacgactgcggagtgtacaagaacttgttattaatgccttattaaagacatgaaagcatacacgttgaaacagtaagaagtatctgtgaagacttcaatttctcaatatgttaagtatattaatatgattgagtggcag

SEQ ID NO: 229 - RNA, 155 nt, synthetic construct
  source 1..155: mol_type = other RNA
catcttaaagcttacgccaatgtgtaggattcgttgcatccgaatttacgcctgtagagtgttataccaaacgtaagtagcttcggcaaaagcgggcacgttgaagcaggaagcaaacaagagttgtgtagacttgtacaatctcttggcaacgg

SEQ ID NO: 230 - RNA, 151 nt, synthetic construct
  source 1..151: mol_type = other RNA
ttaaacaagcgcttatatgtgtaccgaaggctatttcgggaatttacgcctgtggagtgctatacaaactgtagtagcttaggcaaggcagagtacaatgaaacaggaatcttctcagtatggatacatttgaccatattttgagtagcag

SEQ ID NO: 231 - RNA, 186 nt, synthetic construct
  source 1..186: mol_type = other RNA
caccgacaagtcaatgcagatatgtaccgattcgttagtcgggaatttaagcctctggagcgttatatcaaacgtgagtagtctgttcttcgggacggcaaaagcggacgcagtgaatgaggaatggaacgtaaaagttaactttctacggaaggtttatgactttttataagttttcagtaacgg

SEQ ID NO: 232 - RNA, 170 nt, synthetic construct
  source 1..170: mol_type = other RNA
cacattcaagttaatacagatatgtacggattcgttagttcggaatttaagcctatgaagtgtacaagaacttgtgagtagtatctgggtttattcagtacaaaagcatacacgacgaagtaggaatgaaacataaaagtttataactttttataagttttcagtaacgg

SEQ ID NO: 233 - RNA, 155 nt, synthetic construct
  source 1..155: mol_type = other RNA
ccccaataagttaccgctaatctgtaggattcgttgtatccgaatttacgcctgtggagtgtccgatcaaatgcgagtagcttcggccaaagcagacacagagaagcaggaagcaaacaaaagatgtgtagacttttacaatcttttggcaacgg